European Patent Specification EP 3 833 756 B9, published October 4, 2023. Title: EPIMERASE ENZYMES AND THEIR USE. Applicant: Archer Daniels Midland Company. Application EP 19759129.0. The sequence listing filed with the application follows.

SEQUENCE LISTING (100 sequences)

SEQ ID NO: 1 - DNA, 5120 bp, Artificial Sequence
  cassette
taagatgaaaaacgctgacattgactggggacaggtcagtgaccagctagataaagcgaaagataagattacgaaattcatagaatcagatgaaggcaaaaacttcatccagaaagtcattgatttcttcgtatctatctggaatgcgattgtatctatattcaaataagaaaagcgccgaaaaatcggcgtttcttttattgctttacacccgttttaaatggcagatcaagttttacaatatcttcgtatgtttctcgcttcacgactaaatgagcctcaccgttttcgacaaatacaacggcgggtctcggaatacggttataattgttggccatgctgtatccataagcgcctgtacaaaaaacggcaagaagatcgccttcttttacttccggcaggtcaatatcccaaatcagcatatctccgctttcacagcactttccggcaattgataccgttttgtcatgcgcttctccgatcctgttggctgccgcagcttcatatttagcttggtaaagcgcaggacgaatattgtcgttcatgcctccgtctacagccacatattggcggacacccggcacttctttttgagagccaaccgtataaagagttgtgcctgcgtctcccacgagagaacggcccggttcgatccaaatttccggaatgtcaaaaccgtaacgggaagcattttctttcagcatgcttaagttattggtatgactggttttaagcgcaaaaaaagttgctttttcgtacctattaatgtatcgttttagaaaaccgactgtaaaaagtacagtcggcattatctcatattataaaagccagtcattaggcctatctgacaattcctgaatagagttcataaacaatcctgcatgataaccatcacaaacagaatgatgtacctgtaaagatagcggtaaatatattgaattacctttattaatgaattttcctgctgtaataatgggtagaaggtaattactattattattgatatttaagttaaacccagtaaatgaagtccatggaataatagaaagagaaaaagcattttcaggtataggtgttttgggaaacaatttccccgaaccattatatttctctacatcagaaaggtataaatcataaaactctttgaagtcattctttacaggagtccaaataccagagaatgttttagatacaccatcaaaaattgtataaagtggctctaacttatcccaataacctaactctccgtcgctattgtaaccagttctaaaagctgtatttgagtttatcacccttgtcactaagaaaataaatgcagggtaaaatttatatccttcttgttttatgtttcggtataaaacactaatatcaatttctgtggttatactaaaagtcgtttgttggttcaaataatgattaaatatctcttttctcttccaattgtctaaatcaattttattaaagttcatttgatatgcctcctaaatttttatctaaagtgaatttaggaggcttacttgtctgctttcttcattagaatcaatccttttttaaaagtcaatattactgtaacataaatatatattttaaaaatatcccactttatccaattttcgtttgttgaactaatgggtgctttagttgaagaataaagaccacattaaaaaatgtggtcttttgtgtttttttaaaggatttgagcgtagcgaaaaatccttttctttcttatcttgataataagggtaactattgccgatcgtccattccgacagcatcgccagtcactatggcgtgctgctagcgccattcgccattcaggctgcgcaactgttgggaagggcgatcggtgcgggcctcttcgctattacgccagctggcgaaagggggatgtgctgcaaggcgattaagttgggtaacgccagggttttcccagtcacgacgttgtaaaacgacggccagtgaattcgagctcaggccttaactcacattaattgcgttgcgctcactgcccgctttccagtcgggaaacctgtcgtgccagctgcattaatgaatcggccaacgcgcggggagaggcggtttgcgtattgggcgccagggtggtttttcttttcaccagtgagacgggcaacagctgattgcccttcaccgcctggccctgagagagttgcagcaagcggtccacgctggtttgccccagcaggcgaaaatcctgtttgatggtggttgacggcgggatataacatgagctgtcttcggtatcgtcgtatcccactaccgagatatccgcaccaacgcgcagcccggactcggtaatggcgcgcattgcgcccagcgccatctgatcgttggcaaccagcatcgcagtgggaacgatgccctcattcagcatttgcatggtttgttgaaaaccggacatggcactccagtcgccttcccgttccgctatcggctgaatttgattgcgagtgagatatttatgccagccagccagacgcagacgcgccgagacagaacttaatgggcccgctaacagcgcgatttgctggtgacccaatgcgaccagatgctccacgcccagtcgcgtaccgtcttcatgggagaaaataatactgttgatgggtgtctggtcagagacatcaagaaataacgccggaacattagtgcaggcagcttccacagcaatggcatcctggtcatccagcggatagttaatgatcagcccactgacgcgttgcgcgagaagattgtgcaccgccgctttacaggcttcgacgccgcttcgttctaccatcgacaccaccacgctggcacccagttgatcggcgcgagatttaatcgccgcgacaatttgcgacggcgcgtgcagggccagactggaggtggcaacgccaatcagcaacgactgtttgcccgccagttgttgtgccacgcggttgggaatgtaattcagctccgccatcgccgcttccactttttcccgcgttttcgcagaaacgtggctggcctggttcaccacgcgggaaacggtctgataagagacaccggcatactctgcgacatcgtataacgttactggtttcatcaaaatcgtctccctccgtttgaatatttgattgatcgtaaccagatgaagcactctttccactatccctacagtgttatggcttgaacaatcacgaaacaataattggtacgtacgatctttcagccgactcaaacatcaaatcttacaaatgtagtctttgaaagtattacatatgtaagatttaaatgcaaccgttttttcggaaggaaatgatgacctcgtttccaccggaattagcttggtaccaaaggaggtaaggatcactagaaaattttttaaaaaatctcttgacattggaagggagatatgttattataagaattgcggaattgtgagcggataacaattcccatataaaggaggaaggatccatgaataagttaggtgtgcacgcattagtttgggaagcgggttggagtcgtgatgagtgtgctcgtgccatcgcacgcaccgcggaaacgggatttgacttcattgaagtcccagcgttagatccggcaagcattgatgcagagtttactcgcagagagttagaacgccatgggttgggagtaaccttttcgcttggactcgatgcgcaaacagacattagttctggtgatccggaacgcgcagcgcggggtaaagctaaattagacgatgtcttacgtgtagcccgggattgtggagcgactcatgtctgtggaattctctatagtgcatttcaaaaaaatgcagttcctacgacccgtgcgggtgtcgccatggccgcggacattttaggacaggtagctgatactgcagcacaatacggtattactttggggttagaagtcgttaaccgttatgagtcaaatgtattgaacaccgcgtcacagggtgttgaactttgcgagcgtattggtcgtcccaacgtaaaagtgcatttagatacgtatcacatgaatattgaagagagcgatattatgagcgcgatcagagatacgggagacaggctagggtatttccatattggcgattctcatcgtggttacctgggttccggaaacgtcgactttactgccgtatttagggcgctggtattttctggatatacgggaccgattacatttgagtcattctccagtagagtcgtaggacaaccattagagggaattctggcaatttggcgtaatttatgggaagattcccgcgatctagctagtcacgccttagcatatactcgtgtccagttaaaatctgctcaagaagccctaaaacaagccgagcgcagtcgcttaccgtgataacccgggcagcccgcctaatgagcgggcttttttcacgtcacgcgtccatggagatctaagctttcactttttgcttcagggtttcagccgtatggtgatcgagttcgcctgttaatcgaatacaaagcacagattctttgacattcatgtcaattccaaggctcatgctcattcctccttgatatgatcggataatgagtgtttcgatttcgacggaatgaattccttcaccgtgacaaaactagtggtcattcggcataattacttaaattttgtccagtctcccatcgtccgctttaagaatgtgataaacccggctttcttcatatcttcttttgcagcaacaggactttcagcgagtacttctccatcctttttcagaacaagagtgccaagctcttggcctttttgaatcggagcactaatattgtccttcatcttgatttcttttttcacatcgttcatatcctcgccttttttcgtcaatattgaaatcggctcagatgtagtgagttcgataaatttttgtttcccttttttgacctttacttttgctactgtttgatttcgtttatataaaggatgcgtttcatattggctaaaggcgaagtcaagcatttttgtcacttgcgcgtttctttctttaggcgtgctcgctccgaatacaaccgctatggcccgcatgtttccttttttagccgaagcagtcagacaatatttcgcttcgcctgtatagcctgtttttacgccgtctacaccaggat

SEQ ID NO: 2 - DNA, 1925 bp, Artificial Sequence
  cassette
ttattgctttacacccgttttaaatggcagatcaagttttacaatatcttcgtatgtttctcgcttcacgactaaatgagcctcaccgttttcgacaaatacaacggcgggtctcggaatacggttataattgttggccatgctgtatccataagcgcctgtacaaaaaacggcaagaagatcgccttcttttacttccggcaggtcaatatcccaaatcagcatatctccgctttcacagcactttccggcaattgataccgttttgtcatgcgcttctccgatcctgttggctgccgcagcttcatatttagcttggtaaagcgcaggacgaatattgtcgttcatgcctccgtctacagccacatattggcggacacccggcacttctttttgagagccaaccgtataaagagttgtgcctgcgtctcccacgagagaacggcccggttcgatccaaatttccggaatgtcaaaaccgtaacgggaagcattttctttcacagcttcgataattttttcaacgtattcagtggcatgaagcggttcatcatcttccgtataacgaatgccgaaacctcctccaagattcagcaccttggatacaaatgaatatgaatctctccattcgtctagttttttgaagattttttccgctgctaacacaaaaccggccgtatcaaagatttgcgagccgatatggcaatggacacccagcagctgaatgtgttccgattgtaatacttgttcaatggcccgttcagtttgtccgttatgaagatcgaaaccaaactttgaatcttcctggcccgttgtaatgtagtcatgcgtatgcgcttctactccgggcgtgatccgaagaagaacatcgatggagtgacccgtttctttacataggtcttcaagaagcgcgatttcatagaaattatccaccacaatgcagccgatgcggtgctcaagcgccatccgcagttcttccctgctcttattgtttccatgaaagtggatgcgttctgccggaaagcctgctgcaacagccgtatatagctctcctccggatacgacatctaaagaaagtccctcttcctcagcgagctgaatcattgcgactgatgagaatgctttgctcgcatatgccacctgtgctttcagccctgcagaaataaacgcctgcttaaagcttttagcacgctcacgtattaaagccacatcatatacgtaaagaggtgtaccatatttctccgctaaatagagagcatccacacctccgatttctaaatgaccatgttgattttgtctgcttgtgccgtgtaagaacaatgtcattccctctttctccgcttatggatgaaaggacagttttatggactgtcccttcataattaagacatacattatcatactcttcagtcagtttcaatgcgatcactgcccgctttccagtcgggaaacctgtcgtgccagctgcattaatgaatcggccaacgcgcggggagaggcggtttgcgtattgggcgccagggtggtttttcttttcaccagtgagacgggcaacagctgattgcccttcaccgcctggccctgagagagttgcagcaagcggtccacgctggtttgccccagcaggcgaaaatcctgtttgatggtggttgacggcgggatataacatgagctgtcttcggtatcgtcgtatcccactaccgagatatccgcaccaacgcgcagcccggactcggtaatggcgcgcattgcgcccagcgccatctgatcgttggcaaccagcatcgcagtgggaacgatgccctcattcagcatttgcatggtttgttgaaaaccggacatggcactccagtcgccttcccgttccgctatcggctgaatttgattgcgagtgagatatttatgccagccagccagacgcagac

SEQ ID NO: 3 - DNA, 27 bp, Artificial Sequence
  primer
ttattgctttacacccgttttaaatgg

SEQ ID NO: 4 - DNA, 25 bp, Artificial Sequence
  primer
tctcactcgcaatcaaattcagccg

SEQ ID NO: 5 - DNA, 897 bp, Artificial Sequence
  codon optimized sequence for xylose isomerase [Burkholderia multivorans CGD1]
atgaataagttaggtgtgcacgcattagtttgggaagcgggttggagtcgtgatgagtgtgctcgtgccatcgcacgcaccgcggaaacgggatttgacttcattgaagtcccagcgttagatccggcaagcattgatgcagagtttactcgcagagagttagaacgccatgggttgggagtaaccttttcgcttggactcgatgcgcaaacagacattagttctggtgatccggaacgcgcagcgcggggtaaagctaaattagacgatgtcttacgtgtagcccgggattgtggagcgactcatgtctgtggaattctctatagtgcatttcaaaaaaatgcagttcctacgacccgtgcgggtgtcgccatggccgcggacattttaggacaggtagctgatactgcagcacaatacggtattactttggggttagaagtcgttaaccgttatgagtcaaatgtattgaacaccgcgtcacagggtgttgaactttgcgagcgtattggtcgtcccaacgtaaaagtgcatttagatacgtatcacatgaatattgaagagagcgatattatgagcgcgatcagagatacgggagacaggctagggtatttccatattggcgattctcatcgtggttacctgggttccggaaacgtcgactttactgccgtatttagggcgctggtattttctggatatacgggaccgattacatttgagtcattctccagtagagtcgtaggacaaccattagagggaattctggcaatttggcgtaatttatgggaagattcccgcgatctagctagtcacgccttagcatatactcgtgtccagttaaaatctgctcaagaagccctaaaacaagccgagcgcagtcgcttaccgtgataa

SEQ ID NO: 6 - protein, 297 aa, Burkholderia multivorans
MNKLGVHALVWEAGWSRDECARAIARTAETGFDFIEVPALDPASIDAEFTRRELERHGLGVTFSLGLDAQTDISSGDPERAARGKAKLDDVLRVARDCGATHVCGILYSAFQKNAVPTTRAGVAMAADILGQVADTAAQYGITLGLEVVNRYESNVLNTASQGVELCERIGRPNVKVHLDTYHMNIEESDIMSAIRDTGDRLGYFHIGDSHRGYLGSGNVDFTAVFRALVFSGYTGPITFESFSSRVVGQPLEGILAIWRNLWEDSRDLASHALAYTRVQLKSAQEALKQAERSRLP

SEQ ID NO: 7 - DNA, 897 bp, Artificial Sequence
  coding sequence for variant 230323
atgaataagttaggtgtgcacgcattagtttgggaagcgggttggagtcgtgatgagtgtgctcgtgccatcgcacgcaccgcggaaacgggatttgacttcattgaaattccagcgttagatccggcaagcattgatgcagagtttactcgcagagagttagaacgccatgggttgggagtaaccttttcgcttggactcgatgcgcaaacagacattagttctggtgatccggaacgcgcagcggcaggtaaagctaaattagacgatgtcttacgtgtagcccgggattgtggagcgactcatgtctgtggaattctctatagtgcatttcaaaaaaatgcagttcctacgacccgtgcgggtgtcgccatggccgcggacattttaggacaggtagctgatactgcagcacaatacggtattactttggggttagaagtcgttaaccgttatgagacaaatgtattgaacaccgcgtcacagggtgttgaactttgcgagcgtattggtcgtcccaacgtaaaagtgcatttagatacgtatcacatgaatattgaagagagcgatattatgagcgcgatcagagatacgggagacaggctagggtatttccatattggcgattctcatcgtggttacctgggttccggaaacgtcgactttactgccgtatttagggcgctggtattttctggatatacgggaccgattacatttgagtcattctccagtagagtcgtaggacaaccattagagggaattctggcaatttggcgtaatttatgggaagattcccgcgatctagctagtcacgccttagcatatactcgtgtccagttaaaatctgctcaagaagccctaaaacaagccgagcgcagtcgcttaccgtgataa

SEQ ID NO: 8 - protein, 297 aa, Artificial Sequence
  variant 230323
MNKLGVHALVWEAGWSRDECARAIARTAETGFDFIEIPALDPASIDAEFTRRELERHGLGVTFSLGLDAQTDISSGDPERAARGKAKLDDVLRVARDCGATHVCGILYSAFQKNAVPTTRAGVAMAADILGQVADHAAQYGITLGLEVVNRYESNVLNTASQGVELCERIGRPNVKVHLDTYHMNIEESDIMSAIRDTGDRLGYFHIGDSNRGYLGSGNVDFTAVFRALVFSGYTGPITFESFSSRVVGQPLEGILAIWRNLWEDSRDLASHALAYTRVQLKSAQEALKQAERSRLP

SEQ ID NO: 9 - DNA, 897 bp, Artificial Sequence
  coding sequence for variant 230329
atgaataagttaggtgtgcacgcattagtttgggaagcgggttggagtcgtgatgagtgtgctcgtgccatcgcacgcaccgcggaaacgggatttgacttcattgaaattccagcgttagatccggcaagcattgatgcagagtttactcgcagagagttagaacgccatgggttgggagtaaccttttcgcttggactcgatgcgcaaacagacattagttctggtgatccggaacgcgcagcgcggggtaaagctaaattagacgatgtcttacgtgtagcccgggattgtggagcgactcatgtctgtggaattctctatagtgcatttcaaaaaaatgcagttcctacgacccgtgcgggtgtcgccatggccgcggacattttaggacaggtagctgatactgcagcacaatacggtattactttggggttagaagtcgttaaccgttatgagacaaatgtattgaacaccgcgtcacagggtgttgaacttattgagcgtattggtcgtcccaacgtaaaagtgcatttagatacgtatcacatgaatattgaagagagcgatattatgagcgcgatcagagatacgggagacaggctagggtatttccatattggcgattctcatcgtggttacctgggttccggaaacgtcgactttactgccgtatttagggcgctggtattttctggatatacgggaccgattacatttgagtcattctccagtagagtcgtaggacaaccattagagggaattctggcaatttggcgtaatttatgggaagattcccgcgatctagctagtcacgccttagcatatactcgtgtccagttaaaatctgctcaagaagccctaaaacaagccgagcgcagtcgcttaccgtgataa

SEQ ID NO: 10 - protein, 297 aa, Artificial Sequence
  variant 230329
MNKLGVHALVWEAGWSRDECARAIARTAETGFDFIEVPALDPASIDAEFTRRELERHGLGVTFSLGLDAQTDISSGDPERAARGKAKLDDVLRVARDCGATHVAGILYSAFQKNAVPTTRAGVAMAADILGQVADTAAQYGITLGLEVVNRYESHVLNTASQGVELCERIGRPNVKVHLDTYHMNIEESDIMSAIRDTGDRLGYFHIGDSHRGYLGSGNVDFTAVFRALAFSGYTGPITFESFSSRVVGQPLEGILAIWRNLWEDSRDLASHALAYTRVQLKSAQEALKQAERSRLP

SEQ ID NO: 11 - DNA, 897 bp, Artificial Sequence
  coding sequence for variant 230333
atgaataagttaggtgtgcacgcattagtttgggaagcgggttggagtcgtgatgagtgtgctcgtgccatcgcacgcaccgcggaaacgggatttgacttcattgaagtcccagcgttagatccggcaagcattgatgcagagtttactcgcagagagttagaacgccatgggttgggagtaaccttttcgcttggactcgatgcgcaaacagacattagttctggtgatccggaacgcgcagcggcaggtaaagctaaattaaaagatgtcttacgtgtagcccgggattgtggagcgactcatgtctgtggaattctctatagtgcatttcaaaaaaatgcagttcctacgacccgtgcgggtgtcgccatggccgcggacattttaggacaggtagctgatactgcagcacaatacggtattactttggggttagaagtcgttaaccgttatgagtcaaatgtattgaacaccgcgtcacagggtgttgaacttattgagcgtattggtcgtcccaacgtaaaagtgcatttagatacgtatcacatgaatattgaagagagcgatattatgagcgcgatcagagatacgggagacaggctagggtatttccatattggcgattctcatcgtggttacctgggttccggaaacgtcgactttactgccgtatttagggcgctggtattttctggatatacgggaccgattacatttgagtcattctccagtagagtcgtaggacaaccattagagggaattctggcaatttggcgtaatttatgggaagattcccgcgatctagctagtcacgccttagcatatactcgtgtccagttaaaatctgctcaagaagccctaaaacaagccgagcgcagtcgcttaccgtgataa

SEQ ID NO: 12 - protein, 297 aa, Artificial Sequence
  variant 230333
MNKFGVHALVWEAGWSRDECARAIARTAETGFDFIEVPALDPASIDAEFTRRELERHGLGVTFSLGLDAQTDISSGDPERAARGKAKLDDVLRVARDCGATHVCGILYSAFQKNAVPTTRAGVAMAADILGQVADTAAQYGITLGLEVVNRYESNVLNTASQGVELCERIGRPNVKLHLDTYHMNIEESDIMSAIRDTGDRLGYFHIGDSHRGYLGSGNVDFTAVFRALVFSGYTGPITFEPFSSRVVGQPLEGILAIWRNLWEDSRDLASHALAYTRVQLKSAQEALKQAERSRLP

SEQ ID NO: 13 - DNA, 897 bp, Artificial Sequence
  coding sequence for variant 230335
atgaataagttaggtgtgcacgcattagtttgggaagcgggttggagtcgtgatgagtgtgctcgtgccatcgcacgcaccgcggaaacgggatttgacttcattgaagtcccagcgttagatccggcaagcattgatgcagagtttactcgcagagagttagaacgccatgggttgggagtaaccttttcgcttggactcgatgcgcaaacagacattagttctggtgatccggaacgcgcagcggcaggtaaagctaaattagacgatgtcttacgtgtagcccgggattgtggagcgactcatgtctgtggaattctctatagtgcatttcaaaaaaatgcagttcctacgacccgtgcgggtgtcgccatggccgcggacattttaggacaggtagctgatactgcagcacaatacggtattactttggggttagaagtcgttaaccgttatgagacaaatgtattgaacaccgcgtcacagggtgttgaacttattgagcgtattggtcgtcccaacgtaaaagtgcatttagatacgtatcacatgaatattgaagagagcgatattatgagcgcgatcagagatacgggagacaggctagggtatttccatattggcgattctcatcgtggttacctgggttccggaaacgtcgactttactgccgtatttagggcgctggtattttctggatatacgggaccgattacatttgagtcattctccagtagagtcgtaggacaaccattagagggaattctggcaatttggcgtaatttatgggaagattcccgcgatctagctagtcacgccttagcatatactcgtgtccagttaaaatctgctcaagaagccctaaaacaagccgagcgcagtcgcttaccgtgataa

SEQ ID NO: 14 - protein, 297 aa, Artificial Sequence
  variant 230335
MNKLGVHALVWEAGWSRDECARAIARTAETGFDFVEVPALDPASIDAEFTRRELERHGLGVTFSLGLDAQTDISSGDPERAARGKAKLDDVLRVARDCGATHVCGILYSAFQKNAVPTTRAGVAMAADILGQVADTAEQYGITLGLEVVNRYESNVLNTASQGVELCERIGRPNVKVHLDTYHMNIEESDIMSAIRDTGDRLGYFHIGDSHRGYLGSGNLDFTAVFRALVFSGYTGPITFESFSSRVVGQPLEGILAIWRNLWEDSRDLASHALAYTRVQLKSAQEALKQAERSRLP

SEQ ID NO: 15 - DNA, 897 bp, Artificial Sequence
  coding sequence for variant 230338
atgaataagttaggtgtgcacgcattagtttgggaagcgggttggagtcgtgatgagtgtgctcgtgccatcgcacgcaccgcggaaacgggatttgacttcattgaagtcccagcgttagatccggcaagcattgatgcagagtttactcgcagagagttagaacgccatgggttgggagtaaccttttcgcttggactcgatgcgcaaacagacattagttctggtgatccggaacgcgcagcgcggggtaaagctaaattaaaagatgtcttacgtgtagcccgggattgtggagcgactcatgtctgtggaattctctatagtgcatttcaaaaaaatgcagttcctacgacccgtgcgggtgtcgccatggccgcggacattttaggacaggtagctgatactgcagcacaatacggtattactttggggttagaagtcgttaaccgttatgagacaaatgtattgaacaccgcgtcacagggtgttgaacttattgagcgtattggtcgtcccaacgtaaaagtgcatttagatacgtatcacatgaatattgaagagagcgatattatgagcgcgatcagagatacgggagacaggctagggtatttccatattggcgattctcatcgtggttacctgggttccggaaacgtcgactttactgccgtatttagggcgctggtattttctggatatacgggaccgattacatttgagtcattctccagtagagtcgtaggacaaccattagagggaattctggcaatttggcgtaatttatgggaagattcccgcgatctagctagtcacgccttagcatatactcgtgtccagttaaaatctgctcaagaagccctaaaacaagccgagcgcagtcgcttaccgtgataa

SEQ ID NO: 16 - protein, 297 aa, Artificial Sequence
  variant 230338
MNKLGVHALVWEAGWSRDECARAIARTAETGFDFIEVPALDPASIDAEFTRRELERHGLGVTFSLGLDAQTDISSGDPERAARGKAKLKDVLRVARDCGGTHVCGILYSAFQKNAVPTTRAGVAMAADILGQVADTAAQYGITLGLEVVNRYETNLLNTASQGVELIERIGRPNVKVHLDTYHMNIEESDIMSAIRDTGDRLGYFHIGDSHRGYLGSGNVDFTAIFRALVFSGYTGPITFESFSSRVVGQPLEGILAIWRNLWEDSRDLASHALAYTRVQLKSAQEALKQAERSRLP

SEQ ID NO: 17 - DNA, 897 bp, Artificial Sequence
  coding sequence for variant 256407
atgaataagttaggtgtgcacgcattagtttgggaagcgggttggagtcgtgatgagtgtgctcgtgccatcgcacgcaccgcggaaacgggatttgacttcattgaagtcccagcgttagatccggcaagcattgatgcagagtttactcgcagagagttagaacgccatgggttgggagtaaccttttcgcttggactcgatgcgcaaacagacattagttctggtgatccggaacgcgcagcgcggggtaaagctaaattaaaagatgtcttacgtgtagcccgggattgtggagcgactcatgtctgtggaattctctatagtgcactgcaaaaatatgcagttcctacgaccgcagatggtgtcgccatggccgcggacattttaggacaggtagctgatactgcagcacaatacggtattactttggggttagaagtcgttaaccgttatgagacaaatgtattgaacaccgcgtcacagggtgttgaacttattgagcgtattggtcgtcccaacgtaaaagtgcatttagatacgtatcacatgaatattgaagagagcgatattatgagcgcgatcagagatacgggagacaggctagggtatttccatattggcgattctcatcgtggttacctgggttccggaaacgtcgactttactgccgtatttagggcgctggtattttctggatatacgggaccgattacatttgagtcattctccagtagagtcgtaggacaaccattagagggaattctggcaatttggcgtaatttatgggaagattcccgcgatctagctagtcacgccttagcatatactcgtgtccagttaaaatctgctcaagaagccctaaaacaagccgagcgcagtcgcttaccgtgataa

SEQ ID NO: 18 - protein, 297 aa, Artificial Sequence
  variant 256407
MNKLGVHALVWEAGWSRDECARAIARTAETGFDFIEVPALDPASIDAEFTRRELERHGLGVTFSLGLDAQTDISSGDPERAARGKAKLKDVLRVARDCGATHVCGILYSALQKYAVPTTADGVAMAADILGQVADTAAQYGITLGLEVVNRYETNVLNTASQGVELIERIGRPNVKVHLDTYHMNIEESDIMSAIRDTGDRLGYFHIGDSHRGYLGSGNVDFTAVFRALVFSGYTGPITFESFSSRVVGQPLEGILAIWRNLWEDSRDLASHALAYTRVQLKSAQEALKQAERSRLP

SEQ ID NO: 19 - DNA, 897 bp, Artificial Sequence
  coding sequence for variant 230339
atgaataagttaggtgtgcacgcattagtttgggaagcgggttggagtcgtgatgagtgtgctcgtgccatcgcacgcaccgcggaaacgggatttgacttcattgaagtcccagcgttagatccggcaagcattgatgcagagtttactcgcagagagttagaacgccatgggttgggagtaaccttttcgcttggactcgatgcgcaaacagacattagttctggtgatccggaacgcgcagcgcggggtaaagctaaattaaaagatgtcttacgtgtagcccgggattgtggagcgactcatgtctgtggaattctctatagtgcatttcaaaaaaatgcagttcctacgacccgtgcgggtgtcgccatggccgcggacattttaggacaggtagctgatactgcagcacaatacggtattactttggggttagaagtcgttaaccgttatgagacaaatgtattgaacaccgcgtcacagggtgttgaactttgcgagcgtattggtcgtcccaacgtaaaagtgcatttagatacgtatcacatgaatattgaagagagcgatattatgagcgcgatcagagatacgggagacaggctagggtatttccatattggcgattctcatcgtggttacctgggttccggaaacgtcgactttactgccgtatttagggcgctggtattttctggatatacgggaccgattgtttttgagtcattctccagtagagtcgtaggacaaccattagagggaattctggcaatttggcgtaatttatgggaagattcccgcgatctagctagtcacgccttagcatatactcgtgtccagttaaaatctgctcaagaagccctaaaacaagccgagcgcagtcgcttaccgtgataa

SEQ ID NO: 20 - protein, 297 aa, Artificial Sequence
  variant 230339
MNKLGVHALVWEAGWSRDECARAIARTAETGFDFIEVPALDPASIDAEFTRRELERHGLGVTFSLGLDAQTDISSGDPERAARGKAKLDDVLRVARDCGATHVSGILYSAFQKNAVPTTRAEVAMAADILGQVADTAAQYGITLGLEVVNRYETNVLNTASQGVELCERIGRPNVKVHLDTYHMNIEESDIMSAIRDTGDRLGYFHIGDSHRGYLGSGNVDFTAVFRALVFSGYTGPITFESFSSRVVGQPLEGILAIWRNLWEDSRDLASHALAYTRVQLKSAQEALKQAERSRLP

SEQ ID NO: 21 - DNA, 897 bp, Artificial Sequence
  coding sequence for variant 248843
atgaataagttaggtgtgcacgcattagtttgggaagcgggttggagtcgtgatgagtgtgctcgtgccatcgcacgcaccgcggaaacgggatttgacttcattgaagtcccagcgttagatccggcaagcattgatgcagagtttactcgcagagagttagaacgccatgggttgggagtaaccttttcgcttggactcgatgcgcaaacagacattagttctggtgatccggaacgcgcagcgcggggtaaagctaaattaaaagatgtcttacgtgtagcccgggattgtggagcgactcatgtctgtggaattctctatagtgcactgcaaaaaaatgcagttcctacgacccgtgcgggtgtcgccatggccgcggacattttaggacaggtagctgatactgcagcacaatacggtattactttggggttagaagtcgttaaccgttatgagacaaatgtattgaacaccgcgtcacagggtgttgaacttattgagcgtattggtcgtcccaacgtaaaagtgcatttagatacgtatcacatgaatattgaagagagcgatattatgagcgcgatcagagatacgggagacaggctagggtatttccatattggcgattctcatcgtggttacctgggttccggaaacgtcgactttactgccgtatttagggcgctggtattttctggatatacgggaccgattacatttgagtcattctccagtagagtcgtaggacaaccattagagggaattctggcaatttggcgtaatttatgggaagattccgcagatctagctagtcacgccttagcatttactcgtgtccagttaaaatctgctcaagaagccctaaaacaagccgagcgcagtcgcttaccgtgataa

SEQ ID NO: 22 - protein, 297 aa, Artificial Sequence
  variant 248843
MNKLGVHALVWEAGWSRDECARAIARTAETGFDFIEVPALDPASIDAEFTRRELERHGLGVTFSLGLDAQTDISSGDPERAARGKAKLDDVLRVARDCGATHVCGILYSAFQKNAVPTTRAGVAMAADILGQVADTAAQYGITLGLEVVNRYESNVLNTASQGVELCERIGRPNVKVHLDTFHMNIEESDIMSAIRDTGDRLGYFHIGDSHRGYLGSGNVDFTAIFRALVFSGYTGPITIESFSSRVVGQPLEGILAIWRNLWEDSRDLASHALAYTRVQLKSAQEALKQAERSRLP

SEQ ID NO: 23 - DNA, 897 bp, Artificial Sequence
  coding sequence for variant 248867
atgaataagttaggtgtgcacgcattagtttgggaagcgggttggagtcgtgatgagtgtgctcgtgccatcgcacgcaccgcggaaacgggatttgacttcattgaagtcccagcgttagatccggcaagcattgatgcagagtttactcgcagagagttagaacgccatgggttgggagtaaccttttcgcttggactcgatgcgcaaacagacattagttctggtgatccggaacgcgcagcgcggggtaaagctaaattaaaagatgtcttacgtgtagcccgggattgtggagcgactcatgtctgtggaattctctatagtgcatttcaaaaatatgcagttcctacgacccgtgcgggtgtcgccatggccgcggacattttaagacaggtagctgatactgcagcacaatacggtattactttggggttagaagtcgttaaccgttatgagacaaatgtattgaacaccgcgtcacagggtgttgaacttattgagcgtattggtcgtcccaacgtaaaagtgcatttagatacgtatcacatgaatattgaagagagcgatattatgagcgcgatcagagatacgggatcaaggctagggtatttccatattggcgattctcatcgtggttacctgggttccggaaacgtcgactttactgccgtatttagggcgctggtattttctggatatacgggaccgattacatttgagtcattctccagtagagtcgtaggacaaccattagagggaattctggcaatttggcgtaatttatgggaagattcccgcgatctagctagtcacgccttagcatatactcgtgtccagttaaaatctgctcaagaagccctaaaacaagccgagcgcagtcgcttaccgtgataa

SEQ ID NO: 24 - protein, 297 aa, Artificial Sequence
  variant 248867
MNKLGVHALVWEAGWSRDECARAIARTAETGFDFIEVPALDPASIDAEFTRRELERHGLGVTFSLGLDAQTDISSGDPERAARGKAKLDDVLRVARDCGATHVCGILYSAFQKNAVPTTRAGVAMAADILGQVADTAEQYGITLGLEVVNRYESNVLNTASQGVELCERIGRPNVKVHLDTYHMNIEESDIMSAIRDTGDRLGYFHIGDSHRGYLGSGNVDFTAVFRALVFSGYTGPITVESFSSRVVGQPLEGILAIWRNLWEDSRDVASHALAYTRVQLKSAQEALKQAERSRLP

SEQ ID NO: 25 - DNA, 897 bp, Artificial Sequence
  coding sequence for variant 248891
atgaataagttaggtgtgcacgcattagtttgggaagcgggttggagtcgtgatgagtgtgctcgtgccatcgcacgcaccgcggaaacgggatttgacttcattgaagtcccagcgttagatccggcaagcattgatgcagagtttactcgcagagagttagaacgctatgggttgggagtaaccttttcgcttggactcgatgcgcaaacagacattagttctggtgatccggaacgcgcagcgcggggtaaagctaaattaaaagatgtcttacgtgtagcccgggattgtggagcgactcatgtctgtggaattctctatagtgcatttcaaaaaaatgcagttcctacgacccgtgcgggtgtcgccatggccgcggacattttaggacaggtagctgatactgcagcacaatacggtattactttggggttagaagtcgttaaccgttatgagacaaatgtattgaacaccgcgtcacagggtgttgaacttattgagcgtattggtcgtcccaacgtaaaagtgcatttagatacgtatcacatgaatattgaagagagcgatattatgagcgcgatcagagatacgggagacaggctagggtatttccatattggcgaatctcatcgtggttacctgggttccggaaacgtcgactttactgccgtatttagggcgctggtattttctggatatcaaggaccgattacatttgagtcattctccagtagagtcgtaggacaaccattagagggaattctggcaatttggcgtaatttatgggaagattcccgcgatctagctagtcacgccttagcatatactcgtgcacagttaaaatctgctcaagaagccctaaaacaagccgagcgcagtcgcttaccgtgataa

SEQ ID NO: 26 - protein, 297 aa, Artificial Sequence
  variant 248891
MNKLGVHALVWEAGWSRDECARAIARTAETGFDFIEVPALDPASIDAEFTRRELERHGLGVTFSLGLDAQTDISSGDPERAARGKAKLDDVLRVARDCGATHVCGILYSAFQKNAVPTTRAGVAMAADALGQVADTAAQYGITLGLEVVNRYESNVLNTASDGVELCERIGRPNVKVHLDTYHMNIEESDIMSAIRDTGDRLGYFHIGDSHRGYLGSGNVDFTAVFRALVFSGYTGPITFECFSSRVVGQPLEGILAIWRNLWEDSRDLASHALAYTRVQLKSAQEALKQAERSRLP

SEQ ID NO: 27 - DNA, 897 bp, Artificial Sequence
  coding sequence for variant 248907
atgaataagttaggtgtgcacgcattagtttgggaagcgggttggagtcgtgatgagtgtgctcgtgccatcgcacgcaccgcggaaacgggatttgacttcattgaagtcccagcgttagatccggcaagcattgatgcagagtttactcgcagagagttagaacgctatgggttgggagtaaccttttcgcttggactcgatgcgcaaacagacattagttctggtgatccggaacgcgcagcgcggggtaaagctaaattaaaagatgtcttacgtgtagcccgggattgtggagcgactcatgtctgtggaattctctatagtgcatttcaaaaaaatgcagttcctacgacccgtgcgggtgtcgccatggccgcggacattttaagacaggtagctgatactgcagcacaatacggtattactttggggttagaagtcgttaaccgttatgagacaaatgtattgaacaccgcgtcacagggtgttgaacttattgagcgtattggtcgtcccaacgtaaaagtgcatttagatacgtatcacatgaatattgaagagagcgatattatgagcgcgatcagagatacgggagacaggctagggtatttccatattggcgattctcatcgtggttacctgggttccggaaacgtcgactttactgccgtatttagggcgctggtattttctggatatacgggaccgattacatttgagtcattctccagtagagtcgtaggacaaccattagagggaattctggcaatttggcgtaatttatgggaagatggccgcgatctagctagtcacgccttagcatatactcgtgtccagttaaaatctgctcaagaagccctaaaacaagccgagcgcagtcgcttaccgtgataa

SEQ ID NO: 28 - protein, 297 aa, Artificial Sequence
  variant 248907
MNKLGVHALLWEAGWSRDECARAIARTAETGFDFIEIPALDPASIDAEFTRRELERHGLGVTFSLGLDAQTDISSGDPERAARGKAKLDDVLRVARDCGATHVCGILYSAFQKNAVPTTRAGVAMAADILGQVADTAAQYGITLGLEVVNRYESNVLNTASQGVELCERIGRPNVKVHLDTYHMNIEESDIMSAIRDTGDRLGYFHIGDSHRGYLGSGNVDFTAVFRALRFSGYTGPITFESFSSRVVGQPLEGILAIWRNLWEDSRDLASHALAYTRVQLKSAQEALKQAERSRLP

SEQ ID NO: 29 - DNA, 897 bp, Artificial Sequence
  coding sequence for variant 248914
atgaataagttaggtgtgcacgcattagtttgggaagcgggttggagtcgtgatgagtgtgctcgtgccatcgcacgcaccgcggaaacgggatttgacttcattgaagtcccagcgttagatccggcaagcattgatgcagagtttactcgcagagagttagaacgccatgggttgggagtaaccttttcgcttggactcgatgcgcaaacagacattagttctggtgatccggaacgcgcagcgcggggtaaagctaaattaaaagatgtcttacgtgtagcccgggattgtggagcgactcatgtctgtggaattctctatagtgcatttcaaaaatatgcagttcctacgacccgtagaggtgtcgccatggccgcggacattttaggacaggtagctgatactgcagcacaatacggtattatgttggggttagaagtcgttaaccgttatgagacaaatgtattgaacaccgcgtcacagggtgttgaacttattgagcgtattggtcgtcccaacgtaaaagtgcatttagatacgtatcacatgaatattgaagagagcgatattatgagcgcgatcagagatacgggagacaggctagggtatttccatattggcgattctcatcgtggttacctgggttccggaaacgtcgactttactgccgtatttagggcgctggtattttctggatatacgggaccgattacatttgagtcattctccagtagagtcgtaggacaaccattagagggaattctggcaatttggcgtaatttatgggaagattcccgcgatctagctagtcacgccttagcatatactcgtgtccagttaaaatctgctcaagaagccctaaaacaagccgagcgcagtcgcttaccgtgataa

SEQ ID NO: 30 - protein, 297 aa, Artificial Sequence
  variant 248914
MNKLGVHALVWEAGWSRDECARAIARTAETGYDFIELPALDPASIDAEFTRRELERHGLGVTFSLGLDAQTDISSGDPERAARGKAKLDDVLRVARDCGATHVCGILYSAFQKNAVPTTRAGVAMAADILGQVADTAEQYGITLGLEVVNRYESNVLNTASQGVELCERIGRPNVKVHLDTYHMNIEESDIMSAIRDTGDRLGYFHIGDSHRGYLGSGNVDFTAVFRALVFSGYTGPITFESFSSRVVGQPLEGILAIWRNLWEDSRDLASHALAYTRVQLKSAQEALKQAERSRLP

SEQ ID NO: 31 - DNA, 897 bp, Artificial Sequence
  coding sequence for variant 248925
atgaataagttaggtgtgcacgcattagtttgggaagcgggttggagtcgtgatgagtgtgctcgtgccatcgcacgcaccgcggaaacgggatttgacttcattgaagtcccagcgttagatccggcaagcattgatgcagattttactcgcagagagttagaacgccatgggttgggagtaaccttttcgcttggactcgatgcgcaaacagacattagttctggtgatccggaacgcgcagcgcggggtaaagctaaattaaaagatgtcttacgtgtagcccgggattgtggagcgactcatgtctgtggaattctctatagtgcatttcaaaaaaatgcagttcctacgaccgcagcgggtgtcgccatggccgcggacattttaggacaggtagctgatactgcagcacaatacggtattactttggggttagaagtcgttaaccgttatgagacaaatgtattgaacaccgcgtcacagggtgttgaacttattgagcgtattggtcgtcccaacgtaaaagtgcatttagatacgtatcacatgaatattgaagagagcgatattatgagcgcgatcagagatacgggatcaaggctagggtatttccatattggcgattctcatcgtggttacctgggttccggaaacgtcgactttactgccgtatttagggcgctggtattttctggatatacgggaccgattacatttgagtcattctccagtagagtcgtaggacaaccattagagggaattctggcaatttggcgtaatttatgggaagattcccgcgatctagctagtcacgccttagcatatactcgtgtccagttaaaatctgctcaagaagccctaaaacaagccgagcgcagtcgcttaccgtgataa

SEQ ID NO: 32 - protein, 297 aa, Artificial Sequence
  variant 248925
MNKLGVHALVWEAGWSRDECARAIARTAETGFDFIEVPALDPASIDAEFTRRELERHGLGVTFSLGLDAQTDISSGDPERAARGKAKLDDVLRVARDCGATHVCGILYSAFQKNAVPTTRAGVAMAADILGQVADTAEQYGITLGLEVVNRYESNVLNTASQGVELCERIGRPNVKVHLDTYHMNIEESDIMSAIRDTGDRLGYFHIGDSHRGYLGSGNVDFTAVFRALVFSGYTGPITMEAFSSRVVGQPLEGILAIWRNLWEDSRDLASHALAYTRVQLKSAQEALKQAERSRLP

SEQ ID NO: 33 - DNA, 897 bp, Artificial Sequence
  coding sequence for variant 256382
atgaataagttaggtgtgcacgcattagtttgggaagcgggttggagtcgtgatgagtgtgctcgtgccatcgcacgcaccgcggaaacgggatttgacttcattgaagtcccagcgttagatccggcaagcattgatgcagagtttactcgcagagagttagaaaaatatgggttgggagtaaccttttcgcttggactcgatgcgcaaacagacattagttctggtgatccggaacgcgcagcgcggggtaaagctaaattaaaagatgtcttacgtgtagcccgggattgtggagcgactcatgtctgtggaattctctatagtgcactgcaaaaaaatgcagttcctacgacccgtagaggtgtcgccatggccgcggacattttaagacaggtagctgatactgcagcacaatacggtattactttggggttagaagtcgttaaccgttatgagacaaatgtattgaacaccgcgtcacagggtgttgaacttattgagcgtattggtcgtcccaacgtaaaagtgcatttagatacgtatcacatgaatattgaagagagcgatattatgagcgcgatcagagatacgggagacaggctagggtatttccatattggcgattctcatcgtggttacctgggttccggaaacgtcgactttactgccgtatttagggcgctggtattttctggatatacgggaccgattacatttgagtcattctccagtagagtcgtaggacaaccattagagggaattctggcaatttggcgtaatttatgggaagatggccgcgatctagctagtcacgccttagcatatactcgtgtccagttaaaatctgctcaagaagccctaaaacaagccgagcgcagtcgcttaccgtgataa

SEQ ID NO: 34 - protein, 297 aa, Artificial Sequence
  variant 256382
MNKLGVHALVWEAGWSRDECARAIARTAETGYDFIEVPALDPASIDAEFTRRELERHGLGVTFSLGLDAQTDISSGDPERAARGKAKLDDVLRVARDCGATHVCGILYSAFQKNAVPTTRAGVAMAADILGQVADHAAQYGITLGLEVVNRYESNVLNTASQGVELCERIGRPNVKVHLDTYHMNIEESDIMSAIRDTGDRLGYFHIGDSHRGYLGSGNVDFTAVFRALVFSGYTGPITFESFSSRVVGQPLEGILAIWRNLWEDSRDLASHALAYLRVQLKSAQEALKQAERSRLP

SEQ ID NO: 35 - DNA, 897 bp, Artificial Sequence
  coding sequence for variant 256406
atgaataagttaggtgtgcacgcattagtttgggaagcgggttggagtcgtgatgagtgtgctcgtgccatcgcacgcaccgcggaaacgggatttgacttcattgaagtcccagcgttagatccggcaagcattgatgcagagtttactcgcagagagttagaaaaacatgggttgggagtaaccttttcgcttggactcgatgcgcaaacagacgttagttctggtgatccggaacgcgcagcgcggggtaaagctaaattaaaagatgtcttacgtgtagcccgggattgtggagcgactcatgtctgtggaattctctatagtgcatttcaaaaatatgcagttcctacgacccgtagaggtgtcgccatggccgcggacattttaggacaggtagctgatactgcagcacaatacggtattactttggggttagaagtcgttaaccgttatgagacaaatgtattgaacaccgcgtcacagggtgttgaacttattgagcgtattggtcgtcccaacgtaaaagtgcatttagatacgtatcacatgaatattgaagagagcgatattatgagcgcgatcagagatacgggagacaggctagggtatttccatattggcgattctcatcgtggttacctgggttccggaaacgtcgactttactgccgtatttagggcgctggtattttctggatatacgggaccgattacatttgagtcattctccagtagagtcgtaggacaaccattagagggaattctggcaatttggcgtaatttatgggaagatggccgcgatctagctagtcacgccttagcatatactcgtgtccagttaaaatctgctcaagaagccctaaaacaagccgagcgcagtcgcttaccgtgataa

SEQ ID NO: 36 - protein, 297 aa, Artificial Sequence
  variant 256406
MNKLGVHALVWEAGWSRDECARAIARTAETGFDFIEVPALDPASIDAEFTRRELERHGLGVTFSLGLDAQTDISSGDPERAARGKAKLDDVLRVARDCGATHVCGPLYSAFQKNAVPTTRAGVAMAADILGQVADTAAQYGITLGLEVVNRYESNVLNTASQGVELCERIGRPNVKVHLDTYHMNIEESDIMSAIRDTGDRLGYVHIGDSNRGYLGSGNVDFTAVFRALVFSGYTGPITFESFSSRVVGQPLEGILAIWRNLWEDSRDLASHALAYTRVQLKSAQEALKQAERSRLP

SEQ ID NO: 37 - DNA, 897 bp, Artificial Sequence
  coding sequence for variant 255290
atgaataagttaggtgtgcacgcattagtttgggaagcgggttggagtcgtgatgagtgtgctcgtgccatcgcacgcaccgcggaaacgggatttgacttcattgaagtcccagcgttagatccggcaagcattgatgcagagtttactcgcagagagttagaacgccatgggttgggagtaaccttttcgcttggactcgatgcgcaaacagacattagttctggtgatccggaacgcgcagcgcggggtaaagctaaattaaaagatgtcttacgtgtagcccgggattgtggagcgactcatgtctgtggaattctctatagtgcatttcaaaaatatgcagttcctacgacccgtagaggtgtcgccatggccgcggacattttaggacaggtagctgatactgcagcacaatacggtattactttggggttagaagtcgttaaccgttatgagacaaatgtattgaacaccgcgtcacagggtgttgaacttattgagcgtattggtcgtcccaacgtaaaagtgcatttagatacgtatcacatgaatattgaagagagcgatattatgagcgcgatcagagatacgggagacaggctagggtatttccatattggcgattctcatcgtggttacctgggttccggaaacgtcgactttactgccgtatttagggcgctggtattttctggatatacgggaccgattacatttgagtcattctccagtagagtcgtaggacaaccattagagggaattctggcaatttggcgtaatttatgggaagattcccgcgatctagctagtcacgccttagcatatactcgtgtccagttaaaatctgctcaagaagccctaaaacaagccgagcgcagtcgcttaccgtgataa

SEQ ID NO: 38 - protein, 297 aa, Artificial Sequence
  variant 255290
MNKLGVHALVWEAGWSRDECARAIARTAETGFDFIEVPALDPASIDAEFTRRELERHGLGVTFSLGLDAQTDISSGDPERAARGKAKLDDVLRVARDCGATHVCGILYSAFQKNAVPTTRAGVAMAADILGQVADTAAQYGITLGLEVVNRYETYVLNTASQGVELCERIGRPNVKVHLDTYHMNIEESDIMSAIRDTGDRLGYFHIGDSHRGYLGSGNVDFTAVFRALVFSGYTGPITLESFSSRVVGQPLEGILAIWRNLWEDSRDLASHALAYTRVQLKSAQEALKQAERSRLP

SEQ ID NO: 39 - DNA, 897 bp, Artificial Sequence
  coding sequence for variant 257999
atgaataagttaggtgtgcacgcattagtttgggaagcgggttggagtcgtgatgagtgtgctcgtgccatcgcacgcaccgcggaaacgggatttgacttcattgaagtcccagcgttagatccggcaagcattgatgcagagtttactcgcagagagttagaaaaacatgggttgggagtaaccttttcgcttggactcgatgcgcaaacagacattagttctggtgatccggaacgcgcagcgcggggtaaagctaaattaaaagatgtcttacgtgtagcccgggattgtggagcgactcatgtctgtggaattctctatagtgcatttcaaaaatatgcagttcctacgacccgtagaggtgtcgccatggccgcggacattttaggacaggtagctgatactgcagcacaatacggtattactttggggttagaagtcgttaaccgttatgagacaaatgtattgaacaccgcgtcacagggtgttgaacttattgagcgtattggtcgtcccaacgtaaaagtgcatttagatacgtatcacatgaatattgaagagagcgatattatgagcgcgatcagagatacgggagacaggctagggtatttccatattggcgattctcatcgtggttacctgggttccggaaacgtcgactttactgccgtatttagggcgctggtattttctggatatacgggaccgattacatttgagtcattctccagtagagtcgtaggacaaccattagagggaattctggcaatttggcgtaatttatgggaagatggccgcgatctagctagtcacgccttagcatatactcgtgtccagttaaaatctgctcaagaagccctaaaacaagccgagcgcagtcgcttaccgtgataa

SEQ ID NO: 40 - protein, 297 aa, Artificial Sequence
  variant 257999
MNKLGVHALVWEAGWSRDECARAIARTAETGFDFIEVPALDPASIDAEFTRRELEKHGLGVTFSLGLDAQTDISSGDPERAARGKAKLKDVLRVARDCGATHVGGILYSAFQKYAVPTTRRGVAMAADILGQVADTAAQYGITLGLEVVNRYETNVLNTASQGVELIERIGRPNVKVHLDTYHMNIEESDIMSAIRDTGDRLGYFHIGDSHRGYLGSGNLDFTAVFRALVFSGYTGPITIESFSSRVVGQPLEGILAIWRNLWEDGRDLASHALAYTRVQLKSAQEALKQAERSRLP

SEQ ID NO: 41 - DNA, 897 bp, Artificial Sequence
  coding sequence for variant 261731
atgaataagttaggtgtgcacgcattagtttgggaagcgggttggagtcgtgatgagtgtgctcgtgccatcgcacgcaccgcggaaacgggatttgacttcattgaagtcccagcgttagatccggcaagcattgatgcagagtttactcgcagagagttagaaaaacatgggttgggagtaaccttttcgcttggactcgatgcgcaaacagacattagttctggtgatccggaacgcgcagcgcggggtaaagctaaattaaaagatgtcttacgtgtagcccgggattgtggagcgactcatgtctgtggaattctctatagtgcatttcaaaaatatgcagttcctacgaccgcaagaggtgtcgccatggccgcggacattttaggacaggtagctgatactgcagcacaatacggtattactttggggttagaagtcgttaaccgttatgagacaaatgtattgaacaccgcgtcacagggtgttgaacttattgagcgtattggtcgtcccaacgtaaaagtgcatttagatacgtatcacatgaatattgaagagagcgatattatgagcgcgatcagagatacggcagacaggctagggtatttccatattggcgaatctcatcgtggttacctgggttccggaaacgtcgactttactgccgtatttagggcgctggtattttctggatatacgggaccgattacatttgagtcattctccagtagagtcgtaggacaaccattagagggaattctggcaatttggcgtaatttatgggaagatggccgcgatctagctagtcacgccttagcatttactcgtgtccagttaaaatctgctcaagaagccctaaaacaagccgagcgcagtcgcttaccgtgataa

SEQ ID NO: 42 - protein, 297 aa, Artificial Sequence
  variant 261731
MNKLGVHALVWEAGWSRDECARAIARTAETGFDFIEVPALDPASIDAEFTRRELEKHGLGVTFSLGLDAQTDISSGDPERAARGKAKLKDVLRVARDCGATHVCGILYSAFQKYAVPTTARGVAMAADILGQVADHAAQYGITLGLEPVNRYETNVLNTASQGVELIERIGRPNVKVHLDTYHMNIEESDIMSAIRDTADRLGYFHIGESHRGYLGSGNVDFTAVFRALVFSGYTGPITFEPFSSRVVGQPLEGILAIWRNLWEDGRDLASHALAFTRVQLKSAQEALKQAERSRLP

SEQ ID NO: 43 - DNA, 897 bp, Artificial Sequence
  coding sequence for variant 261732
atgaataagttaggtgtgcacgcattagtttgggaagcgggttggagtcgtgatgagtgtgctcgtgccatcgcacgcaccgcggaaacgggatttgacttcattgaagtcccagcgttagatccggcaagcattgatgcagagtttactcgcagagagttagaaaaacatgggttgggagtaaccttttcgcttggactcgatgcgcaatgcgacattagttctggtgatccggaacgcgcagcgcggggtaaagctaaattaaaagatgtcttacgtgtagcccgggattgtggagcgactcatgtctgtggaattctctatagtgcatttcaaaaatatgcagttcctacgaccgcaagaggtgtcgccatggccgcggacattttaggacaggtagctgatactgcagcacaatacggtattactttggggttagaagtcgttaaccgttatgagacaaatgtattgaacaccgcgtcacagggtgttgaacttattgagcgtattggtcgtcccaacgtaaaagtgcatttagatacgtatcacatgaatattgaagagagcgatattatgagcgcgatcagagatacgggagacaggctagggtatttccatattggcgaatctcatcgtggttacctgggttccggaaacgtcgactttactgccgtatttagggcgctggtattttctggatatacgggaccgattacatttgagtcattctccagtagagtcgtaggacaaccattagagggaattctggcaatttggcgtaatttatgggaagatggccgcgatctagctagtcacgccttagcatttactcgtgtccagttaaaatctgctcaagaagccctaaaacaagccgagcgcagtcgcttaccgtgataa

SEQ ID NO: 44 - protein, 297 aa, Artificial Sequence
  variant 261732
MNKLGVHALLWEAGWSRDECARAIARTAETGFDFIEVPALDPASIDAEFTRRELEKHGLGVTFSLGLDAQCDISSGDPERAARGKAKLKDVLRVARDCGATHVCGILYSAFQKYAVPTTARGVAMAADILGQVADTAAQYGITLGLEPVNRYETNVLNTASQGVELIERIGRPNVKVHLDTYHMNIEESDIMSAIRDTGDRLGYVHIGESHRGYLGSGNVDFTAVFRALVFSGYTGPITFESFSSRVVGQPLEGILAIWRNLWEDGRDLASHALAFTRVQLKSAQEALKQAERSRLP

SEQ ID NO: 45 - DNA, 897 bp, Artificial Sequence
  coding sequence for variant 261733
atgaataagttaggtgtgcacgcattagtttgggaagcgggttggagtcgtgatgagtgtgctcgtgccatcgcacgcaccgcggaaacgggatttgacttcattgaagtcccagcgttagatccggcaagcattgatgcagagtttactcgcagagagttagaaaaacatgggttgggagtaaccttttcgcttggactcgatgcgcaatgcgacattagttctggtgatccggaacgcgcagcgcggggtaaagctaaattaaaagatgtcttacgtgtagcccgggattgtggagcgactcatgtctgtggaattctctatagtgcatttcaaaaatatgcagttcctacgaccgcaagaggtgtcgccatggccgcggacattttaggacaggtagctgatactgcagcacaatacggtattactttggggttagaagtcgttaaccgttatgagacaaatgtattgaacaccgcgtcacagggtgttgaacttattgagcgtattggtcgtcccaacgtaaaagtgcatttagatacgtatcacatgaatattgaagagagcgatattatgagcgcgatcagagatacggcagacaggctagggtatttccatattggcgaatctcatcgtggttacctgggttccggaaacgtcgactttactgccgtatttagggcgctggtattttctggatatacgggaccgattacatttgagtcattctccagtagagtcgtaggacaaccattagagggaattctggcaatttggcgtaatttatgggaagatggccgcgatctagctagtcacgccttagcatatactcgtgtccagttaaaatctgctcaagaagccctaaaacaagccgagcgcagtcgcttaccgtgataa

SEQ ID NO: 46 - protein, 297 aa, Artificial Sequence
  variant 261733
MNKLGVHALVWEAGWSRDECARAIARTAETGFDFIEVPALDPASIDAEFTRRELEKHGLGVTFSLGLDAQCDISSGDPERAARGKAKLKDVLRVARDCGATHVCGILYSAFQKYAVPTTARGVAMAADALGQVADTAAQYGITLGLEVVNRYETNVLNTASQGVELIERIGRPNVKVHLDTYHMNIEESDIMSAIRDTADRLGYFHIGESHRGYLGSGNVDFTAIFRALVFSGYTGPITFEPFSSRVVGQPLEGILAIWRNLWEDGRDLASHALAYTRVQLKSAQEALKQAERSRLP

SEQ ID NO: 47 - DNA, 897 bp, Artificial Sequence
  coding sequence for variant 261734
atgaataagttaggtgtgcacgcattagtttgggaagcgggttggagtcgtgatgagtgtgctcgtgccatcgcacgcaccgcggaaacgggatttgacttcattgaagtcccagcgttagatccggcaagcattgatgcagagtttactcgcagagagttagaaaaacatgggttgggagtaaccttttcgcttggactcgatgcgcaatgcgacattagttctggtgatccggaacgcgcagcgcggggtaaagctaaattaaaagatgtcttacgtgtagcccgggattgtggagcgactcatgtctgtggaattctctatagtgcatttcaaaaatatgcagttcctacgaccgcaagaggtgtcgccatggccgcggacattttaggacaggtagctgatactgcagcacaatacggtattactttggggttagaagtcgttaaccgttatgagacaaatgtattgaacaccgcgtcacagggtgttgaacttattgagcgtattggtcgtcccaacgtaaaagtgcatttagatacgtatcacatgaatattgaagagagcgatattatgagcgcgatcagagatacggcagacaggctagggtatttccatattggcgattctcatcgtggttacctgggttccggaaacgtcgactttactgccgtatttagggcgctggtattttctggatatacgggaccgattacatttgagtcattctccagtagagtcgtaggacaaccattagagggaattctggcaatttggcgtaatttatgggaagatggccgcgatctagctagtcacgccttagcatttactcgtgtccagttaaaatctgctcaagaagccctaaaacaagccgagcgcagtcgcttaccgtgataa

SEQ ID NO: 48 - protein, 297 aa, Artificial Sequence
  variant 261734
MNKLGVHALVWEAGWSRDECARAIARTAETGFDFIEVPALDPASIDAEFTRRELEKHGLGVTFSLGLDAQCDISSGDPERAARGKAKLKDVLRVARDCGATHVCGILYSAFQKYAVPTTARGVAMAADILGQVADTAAQYGITLGLEVVNRYETNVLNTASQGVELIERIGRPNVKVHLDTYHMNIEESDIMSAIRDTADRLGYFHIGDSHRGYLGSGNVDFTAVFRALVFSGYTGPITFESFSSRVVGQPLEGILAIWRNLWEDGRDLASHALAFTRVQLKSAQEALKQAERSRLP

SEQ ID NO: 49 - DNA, 897 bp, Artificial Sequence
  coding sequence for variant 261735
atgaataagttaggtgtgcacgcattagtttgggaagcgggttggagtcgtgatgagtgtgctcgtgccatcgcacgcaccgcggaaacgggatttgacttcattgaagtcccagcgttagatccggcaagcattgatgcagagtttactcgcagagagttagaaaaacatgggttgggagtaaccttttcgcttggactcgatgcgcaatgcgacattagttctggtgatccggaacgcgcagcgcggggtaaagctaaattaaaagatgtcttacgtgtagcccgggattgtggagcgactcatgtctgtggaattctctatagtgcatttcaaaaatatgcagttcctacgacccgtagaggtgtcgccatggccgcggacattttaggacaggtagctgatactgcagcacaatacggtattactttggggttagaagtcgttaaccgttatgagacaaatgtattgaacaccgcgtcacagggtgttgaacttattgagcgtattggtcgtcccaacgtaaaagtgcatttagatacgtatcacatgaatattgaagagagcgatattatgagcgcgatcagagatacggcagacaggctagggtatttccatattggcgaatctcatcgtggttacctgggttccggaaacgtcgactttactgccgtatttagggcgctggtattttctggatatacgggaccgattacatttgagtcattctccagtagagtcgtaggacaaccattagagggaattctggcaatttggcgtaatttatgggaagatggccgcgatctagctagtcacgccttagcatttactcgtgtccagttaaaatctgctcaagaagccctaaaacaagccgagcgcagtcgcttaccgtgataa

SEQ ID NO: 50 - protein, 297 aa, Artificial Sequence
  variant 261735
MNKLGVHALVWEAGWSRDECARAIARTAETGFDFIEVPALDPASIDAEFTRRELEKHGLGVTFSLGLDAQCDISSGDPERAARGKAKLKDVLRVARDCGATHVSGILYSAFQKYAVPTTRRGVAMAADILGQVADTAEQYGITLGLEVVNRYETNVLNTASQGVELIERIGRPNVKVHLDTYHMNIEESDIMSAIRDTADRLGYFHIGESHRGYLGSGNVDFTAVFRALVFSGYTGPITLESFSSRVVGQPLEGILAIWRNLWEDGRDLASHALAFTRVQLKSAQEALKQAERSRLP

SEQ ID NO: 51 - DNA, 897 bp, Artificial Sequence
  coding sequence for variant 261736
atgaataagttaggtgtgcacgcattagtttgggaagcgggttggagtcgtgatgagtgtgctcgtgccatcgcacgcaccgcggaaacgggatttgacttcattgaagtcccagcgttagatccggcaagcattgatgcagagtttactcgcagagagttagaaaaacatgggttgggagtaaccttttcgcttggactcgatgcgcaaacagacattagttctggtgatccggaacgcgcagcgcggggtaaagctaaattaaaagatgtcttacgtgtagcccgggattgtggagcgactcatgtctgtggaattctctatagtgcatttcaaaaatatgcagttcctacgaccgcaagaggtgtcgccatggccgcggacattttaggacaggtagctgatactgcagcacaatacggtattactttggggttagaagtcgttaaccgttatgagacaaatgtattgaacaccgcgtcacagggtgttgaacttattgagcgtattggtcgtcccaacgtaaaagtgcatttagatacgtatcacatgaatattgaagagagcgatattatgagcgcgatcagagatacgggagacaggctagggtatttccatattggcgaatctcatcgtggttacctgggttccggaaacgtcgactttactgccgtatttagggcgctggtattttctggatatacgggaccgattacatttgagtcattctccagtagagtcgtaggacaaccattagagggaattctggcaatttggcgtaatttatgggaagatggccgcgatctagctagtcacgccttagcatttactcgtgtccagttaaaatctgctcaagaagccctaaaacaagccgagcgcagtcgcttaccgtgataa

SEQ ID NO: 52 - protein, 297 aa, Artificial Sequence
  variant 261736
MNKLGVHALVWEAGWSRDECARAIARTAETGFDFIEVPALDPASIDAEFTRRELEKHGLGVTFSLGLDAQTDISSGDPERAARGKAKLKDVLRVARDCGATHVCGPLYSAFQKYAVPTTARGVAMAADILGQVADTAAQYGITLGLEVVNRYETNVLNTASQGVELIERIGRPNVKVLLDTYHMNIEESDIMSAIRDTGDRLGYFHIGESHRGYLGSGNIDFTAVFRALVFSGYTGPITFESFSSRVVGQPLEGILAIWRNLWEDGRDLASHALAFTRVQLKSAQEALKQAERSRLP

SEQ ID NO: 53 - DNA, 897 bp, Artificial Sequence
  coding sequence for variant 261737
atgaataagttaggtgtgcacgcattagtttgggaagcgggttggagtcgtgatgagtgtgctcgtgccatcgcacgcaccgcggaaacgggatttgacttcattgaagtcccagcgttagatccggcaagcattgatgcagagtttactcgcagagagttagaaaaacatgggttgggagtaaccttttcgcttggactcgatgcgcaaacagacattagttctggtgatccggaacgcgcagcgcggggtaaagctaaattaaaagatgtcttacgtgtagcccgggattgtggagcgactcatgtctgtggaattctctatagtgcatttcaaaaatatgcagttcctacgaccgcaagaggtgtcgccatggccgcggacattttaggacaggtagctgatactgcagcacaatacggtattactttggggttagaagtcgttaaccgttatgagacaaatgtattgaacaccgcgtcacagggtgttgaacttattgagcgtattggtcgtcccaacgtaaaagtgcatttagatacgtatcacatgaatattgaagagagcgatattatgagcgcgatcagagatacggcagacaggctagggtatttccatattggcgaatctcatcgtggttacctgggttccggaaacgtcgactttactgccgtatttagggcgctggtattttctggatatacgggaccgattacatttgagtcattctccagtagagtcgtaggacaaccattagagggaattctggcaatttggcgtaatttatgggaagatggccgcgatctagctagtcacgccttagcatatactcgtgtccagttaaaatctgctcaagaagccctaaaacaagccgagcgcagtcgcttaccgtgataa

SEQ ID NO: 54 - protein, 297 aa, Artificial Sequence
  variant 261737
MNKLGVHALVWEAGWSRDECARAIARTAETGFDFIEVPALDPASIDAEFTRRELEKHGLGVTFSLGLDAQTDISSGDPERAARGKAKLKDVLRVARDCGATHVSGILYSAFQKYAVPTTARGVAMAADILGQVADTAAQYGITLGLEVVNRFETNLLNTASQGVELIERIGRPNVKVHLDTYHMNIEESDIMSAIRDTADRLGYFHIGESHRGYLGSGNVDFTAVFRALVFSGYTGPITFESFSSRVVGQPLEGILAIWRNLWEDGRDLASHALAYTRVQLKSAQEALKQAERSRLP

SEQ ID NO: 55 - DNA, 897 bp, Artificial Sequence
  coding sequence for variant 261738
atgaataagttaggtgtgcacgcattagtttgggaagcgggttggagtcgtgatgagtgtgctcgtgccatcgcacgcaccgcggaaacgggatttgacttcattgaagtcccagcgttagatccggcaagcattgatgcagagtttactcgcagagagttagaaaaacatgggttgggagtaaccttttcgcttggactcgatgcgcaatgcgacattagttctggtgatccggaacgcgcagcgcggggtaaagctaaattaaaagatgtcttacgtgtagcccgggattgtggagcgactcatgtctgtggaattctctatagtgcatttcaaaaatatgcagttcctacgaccgcaagaggtgtcgccatggccgcggacattttaggacaggtagctgatactgcagcacaatacggtattactttggggttagaagtcgttaaccgttatgagacaaatgtattgaacaccgcgtcacagggtgttgaacttattgagcgtattggtcgtcccaacgtaaaagtgcatttagatacgtatcacatgaatattgaagagagcgatattatgagcgcgatcagagatacgggagacaggctagggtatttccatattggcgaatctcatcgtggttacctgggttccggaaacgtcgactttactgccgtatttagggcgctggtattttctggatatacgggaccgattacatttgagtcattctccagtagagtcgtaggacaaccattagagggaattctggcaatttggcgtaatttatgggaagatggccgcgatctagctagtcacgccttagcatatactcgtgtccagttaaaatctgctcaagaagccctaaaacaagccgagcgcagtcgcttaccgtgataa

SEQ ID NO: 56 - protein, 297 aa, Artificial Sequence
  variant 261738
MNKIGVHALVWEAGWSRDECARAIARTAETGFDFIEVPALDPASIDAEFTRRELEKHGLGVTFSLGLDAQCDISSGDPERAARGKAKLKDVLRVARDCGATHVCGILYSAFQKYAVPTTAREVAMAADILGQVADTAAQYGITLGLEPVNRYETNVLNTASQGVELIERIGRPNVKVHLDTYHMNIEESDIMSAIRDTGDRLGYFHIGESHRGYLGSGNVDFTAVFRALVFSGYTGPITFESFSSRVVGQPLEGILAIWRNLWEDGRDLASHALAYTRVQLKSAQEALKQAERSRLP

SEQ ID NO: 57 - DNA, 897 bp, Artificial Sequence
  coding sequence for variant 261739
atgaataagttaggtgtgcacgcattagtttgggaagcgggttggagtcgtgatgagtgtgctcgtgccatcgcacgcaccgcggaaacgggatttgacttcattgaagtcccagcgttagatccggcaagcattgatgcagagtttactcgcagagagttagaaaaacatgggttgggagtaaccttttcgcttggactcgatgcgcaaacagacattagttctggtgatccggaacgcgcagcgcggggtaaagctaaattaaaagatgtcttacgtgtagcccgggattgtggagcgactcatgtctgtggaattctctatagtgcatttcaaaaatatgcagttcctacgacccgtagaggtgtcgccatggccgcggacattttaggacaggtagctgatactgcagcacaatacggtattactttggggttagaagtcgttaaccgttatgagacaaatgtattgaacaccgcgtcacagggtgttgaacttattgagcgtattggtcgtcccaacgtaaaagtgcatttagatacgtatcacatgaatattgaagagagcgatattatgagcgcgatcagagatacggcagacaggctagggtatttccatattggcgaatctcatcgtggttacctgggttccggaaacgtcgactttactgccgtatttagggcgctggtattttctggatatacgggaccgattacatttgagtcattctccagtagagtcgtaggacaaccattagagggaattctggcaatttggcgtaatttatgggaagatggccgcgatctagctagtcacgccttagcatttactcgtgtccagttaaaatctgctcaagaagccctaaaacaagccgagcgcagtcgcttaccgtgataa

SEQ ID NO: 58 - protein, 297 aa, Artificial Sequence
  variant 261739
MNKLGVHALVWEAGWSRDECARAIARTAETGFDFIEVPALDPASIDAEFTRRELEKHGLGVTFSLGLDAQTDISSGDPERAARGKAKLKDVLRVARDCGATHVGGILYSAFQKYAVPTTRRGVAMAADILGQVADTAAQYGITLGLEVVNRYETNVLNTASDGVELIERIGRPNVKVLLDTYHMNIEESDIMSAIRDTADRLGYFHIGESHRGYLGSGNVDFTAVFRALVFSGYTGPITFESFSSRVVGQPLEGILAIWRNLWEDGRDLASHALAFTRVQLKSAQEALKQAERSRLP

SEQ ID NO: 59 - DNA, 897 bp, Artificial Sequence
  coding sequence for variant 261740
atgaataagttaggtgtgcacgcattagtttgggaagcgggttggagtcgtgatgagtgtgctcgtgccatcgcacgcaccgcggaaacgggatttgacttcattgaagtcccagcgttagatccggcaagcattgatgcagagtttactcgcagagagttagaaaaacatgggttgggagtaaccttttcgcttggactcgatgcgcaatgcgacattagttctggtgatccggaacgcgcagcgcggggtaaagctaaattaaaagatgtcttacgtgtagcccgggattgtggagcgactcatgtctgtggaattctctatagtgcatttcaaaaatatgcagttcctacgacccgtagaggtgtcgccatggccgcggacattttaggacaggtagctgatactgcagcacaatacggtattactttggggttagaagtcgttaaccgttatgagacaaatgtattgaacaccgcgtcacagggtgttgaacttattgagcgtattggtcgtcccaacgtaaaagtgcatttagatacgtatcacatgaatattgaagagagcgatattatgagcgcgatcagagatacgggagacaggctagggtatttccatattggcgaatctcatcgtggttacctgggttccggaaacgtcgactttactgccgtatttagggcgctggtattttctggatatacgggaccgattacatttgagtcattctccagtagagtcgtaggacaaccattagagggaattctggcaatttggcgtaatttatgggaagatggccgcgatctagctagtcacgccttagcatttactcgtgtccagttaaaatctgctcaagaagccctaaaacaagccgagcgcagtcgcttaccgtgataa

SEQ ID NO: 60 - protein, 297 aa, Artificial Sequence
  variant 261740
MNKLGVHALVWEAGWSRDECARAIARTAETGFDFIEIPALDPASIDAEFTRRELEKHGLGVTFSLGLDAQCDISSGDPERAARGKAKLKDVLRVARDCGATHVSGILYSAFQKYAVPTTRRGVAMAADILGQVADTAAQYGITLGLEVVNRYETNVLNTASQGVELIERIGRPNVKVHLDTYHMNIEESDIMSAIRDTGDRLGYFHIGESHRGYLGSGNVDFTAVFRALVFSGYTGPLTFESFSSRVVGQPLEGILAIWRNLWEDGRDLASHALAFTRVQLKSAQEALKQAERSRLP

SEQ ID NO: 61 - DNA, 897 bp, Artificial Sequence
  coding sequence for variant 261741
atgaataagttaggtgtgcacgcattagtttgggaagcgggttggagtcgtgatgagtgtgctcgtgccatcgcacgcaccgcggaaacgggatttgacttcattgaagtcccagcgttagatccggcaagcattgatgcagagtttactcgcagagagttagaaaaacatgggttgggagtaaccttttcgcttggactcgatgcgcaatgcgacattagttctggtgatccggaacgcgcagcgcggggtaaagctaaattaaaagatgtcttacgtgtagcccgggattgtggagcgactcatgtctgtggaattctctatagtgcatttcaaaaatatgcagttcctacgacccgtagaggtgtcgccatggccgcggacattttaggacaggtagctgatactgcagcacaatacggtattactttggggttagaagtcgttaaccgttatgagacaaatgtattgaacaccgcgtcacagggtgttgaacttattgagcgtattggtcgtcccaacgtaaaagtgcatttagatacgtatcacatgaatattgaagagagcgatattatgagcgcgatcagagatacggcagacaggctagggtatttccatattggcgattctcatcgtggttacctgggttccggaaacgtcgactttactgccgtatttagggcgctggtattttctggatatacgggaccgattacatttgagtcattctccagtagagtcgtaggacaaccattagagggaattctggcaatttggcgtaatttatgggaagatggccgcgatctagctagtcacgccttagcatttactcgtgtccagttaaaatctgctcaagaagccctaaaacaagccgagcgcagtcgcttaccgtgataa

SEQ ID NO: 62 - protein, 297 aa, Artificial Sequence
  variant 261741
MNKFGVHALVWEAGWSRDECARAIARTAETGFDFIEVPALDPASIDAEFTRRELEKHGLGVTFSLGLDAQCDISSGDPERAARGKAKLKDVLRVARDCGATHVCGILYSAFQKYAVPTTRRGVAMAADILGQVADTAAQYGITLGLEVVNRYETNVLNTASQGVELIERIGRPNVKVHLDTFHMNIEESDIMSAIRDTADRLGYFHIGDSHRGYLGSGNVDFTAVFRALRFSGYTGPITFESFSSRVVGQPLEGILAIWRNLWEDGRDLASHALAFTRVQLKSAQEALKQAERSRLP

SEQ ID NO: 63 - DNA, 897 bp, Artificial Sequence
  coding sequence for variant 261742
atgaataagttaggtgtgcacgcattagtttgggaagcgggttggagtcgtgatgagtgtgctcgtgccatcgcacgcaccgcggaaacgggatttgacttcattgaagtcccagcgttagatccggcaagcattgatgcagagtttactcgcagagagttagaaaaacatgggttgggagtaaccttttcgcttggactcgatgcgcaaacagacattagttctggtgatccggaacgcgcagcgcggggtaaagctaaattaaaagatgtcttacgtgtagcccgggattgtggagcgactcatgtctgtggaattctctatagtgcatttcaaaaatatgcagttcctacgaccgcaagaggtgtcgccatggccgcggacattttaggacaggtagctgatactgcagcacaatacggtattactttggggttagaagtcgttaaccgttatgagacaaatgtattgaacaccgcgtcacagggtgttgaacttattgagcgtattggtcgtcccaacgtaaaagtgcatttagatacgtatcacatgaatattgaagagagcgatattatgagcgcgatcagagatacggcagacaggctagggtatttccatattggcgattctcatcgtggttacctgggttccggaaacgtcgactttactgccgtatttagggcgctggtattttctggatatacgggaccgattacatttgagtcattctccagtagagtcgtaggacaaccattagagggaattctggcaatttggcgtaatttatgggaagatggccgcgatctagctagtcacgccttagcatttactcgtgtccagttaaaatctgctcaagaagccctaaaacaagccgagcgcagtcgcttaccgtgataa

SEQ ID NO: 64 - protein, 297 aa, Artificial Sequence
  variant 261742
MNKLGVHALVWEAGWSRDECARAIARTAETGFDFIELPALDPASIDAEFTRRELEKHGLGVTFSLGLDAQTDISSGDPERAARGKAKLKDVLRVARDCGATHVGGILYSAFQKYAVPTTARGVAMAADILGQVADTAAQYGITLALEVVNRYETNVLNTASQGVELIERIGRPNVKVHLDTYHMNIEESDIMSAIRDTADRLGYFHIGDSHRGYLGSGNVDFTAVFRALVFSGYTGPITFESFSSRVVGQPLEGILAIWRNLWEDGRDLASHALAFTRVQLKSAQEALKQAERSRLP

SEQ ID NO: 65 - DNA, 897 bp, Artificial Sequence
  coding sequence for variant 261743
atgaataagttaggtgtgcacgcattagtttgggaagcgggttggagtcgtgatgagtgtgctcgtgccatcgcacgcaccgcggaaacgggatttgacttcattgaagtcccagcgttagatccggcaagcattgatgcagagtttactcgcagagagttagaaaaacatgggttgggagtaaccttttcgcttggactcgatgcgcaatgcgacattagttctggtgatccggaacgcgcagcgcggggtaaagctaaattaaaagatgtcttacgtgtagcccgggattgtggagcgactcatgtctgtggaattctctatagtgcatttcaaaaatatgcagttcctacgaccgcaagaggtgtcgccatggccgcggacattttaggacaggtagctgatactgcagcacaatacggtattactttggggttagaagtcgttaaccgttatgagacaaatgtattgaacaccgcgtcacagggtgttgaacttattgagcgtattggtcgtcccaacgtaaaagtgcatttagatacgtatcacatgaatattgaagagagcgatattatgagcgcgatcagagatacgggagacaggctagggtatttccatattggcgattctcatcgtggttacctgggttccggaaacgtcgactttactgccgtatttagggcgctggtattttctggatatacgggaccgattacatttgagtcattctccagtagagtcgtaggacaaccattagagggaattctggcaatttggcgtaatttatgggaagatggccgcgatctagctagtcacgccttagcatttactcgtgtccagttaaaatctgctcaagaagccctaaaacaagccgagcgcagtcgcttaccgtgataa

SEQ ID NO: 66 - protein, 297 aa, Artificial Sequence
  variant 261743
MNKLGVHALVWEAGWSRDECARAIARTAETGFDFIEVPALDPASIDAEFTRRELEKHGLGVTFSLGLDAQCDISSPDPERAARGKAKLKDVLRVARDCGATHVCGILYSAFQKYAVPTTARGVAMAADILGQVADTAAQYGITLGLEVVNRYETNVLNTASQGVELIERIGRPNVKVHLDTYHMNIEESDIMSAIRDTGDRLGYFHIGDSHRGYLGSGNVDWTAVFRALVFSGYTGPITFESFSSRVVGQPLEGILAIWRNLWEDGRDLASHALAFTRVQLKSAQEALKQAERSRLP

SEQ ID NO: 67 - DNA, 897 bp, Artificial Sequence
  coding sequence for variant 261744
atgaataagttaggtgtgcacgcattagtttgggaagcgggttggagtcgtgatgagtgtgctcgtgccatcgcacgcaccgcggaaacgggatttgacttcattgaagtcccagcgttagatccggcaagcattgatgcagagtttactcgcagagagttagaaaaacatgggttgggagtaaccttttcgcttggactcgatgcgcaatgcgacattagttctggtgatccggaacgcgcagcgcggggtaaagctaaattaaaagatgtcttacgtgtagcccgggattgtggagcgactcatgtctgtggaattctctatagtgcatttcaaaaatatgcagttcctacgacccgtagaggtgtcgccatggccgcggacattttaggacaggtagctgatactgcagcacaatacggtattactttggggttagaagtcgttaaccgttatgagacaaatgtattgaacaccgcgtcacagggtgttgaacttattgagcgtattggtcgtcccaacgtaaaagtgcatttagatacgtatcacatgaatattgaagagagcgatattatgagcgcgatcagagatacggcagacaggctagggtatttccatattggcgaatctcatcgtggttacctgggttccggaaacgtcgactttactgccgtatttagggcgctggtattttctggatatacgggaccgattacatttgagtcattctccagtagagtcgtaggacaaccattagagggaattctggcaatttggcgtaatttatgggaagatggccgcgatctagctagtcacgccttagcatatactcgtgtccagttaaaatctgctcaagaagccctaaaacaagccgagcgcagtcgcttaccgtgataa

SEQ ID NO: 68 - protein, 297 aa, Artificial Sequence
  variant 261744
MNKLGVHALVWEAGWSRDECARAIARTAETGFDFIEVPALDPASIDAEFTRRELEKHGLGVTFSLGLDAQCDISSGDPERAARGKAKLKDVLRVARDCGATHVCGPLYSAFQKYAVPTTRRGVAMAADILGQVADTAAQYGITLGLEVLNRYETNVLNTASEGVELIERIGRPNVKVHLDTYHMNIEESDIMSAIRDTGDRLGYFHIGESHRGYLGSGNVDFTAVFRALVFSGYTGPITFESFSSRVVGQPLEGILAIWRNLWEDGRDLASHALAYTRVQLKSAQEALKQAERSRLP

SEQ ID NO: 69 - DNA, 897 bp, Artificial Sequence
  coding sequence for variant 261745
atgaataagttaggtgtgcacgcattagtttgggaagcgggttggagtcgtgatgagtgtgctcgtgccatcgcacgcaccgcggaaacgggatttgacttcattgaagtcccagcgttagatccggcaagcattgatgcagagtttactcgcagagagttagaaaaacatgggttgggagtaaccttttcgcttggactcgatgcgcaatgcgacattagttctggtgatccggaacgcgcagcgcggggtaaagctaaattaaaagatgtcttacgtgtagcccgggattgtggagcgactcatgtctgtggaattctctatagtgcatttcaaaaatatgcagttcctacgaccgcaagaggtgtcgccatggccgcggacattttaggacaggtagctgatactgcagcacaatacggtattactttggggttagaagtcgttaaccgttatgagacaaatgtattgaacaccgcgtcacagggtgttgaacttattgagcgtattggtcgtcccaacgtaaaagtgcatttagatacgtatcacatgaatattgaagagagcgatattatgagcgcgatcagagatacggcagacaggctagggtatttccatattggcgattctcatcgtggttacctgggttccggaaacgtcgactttactgccgtatttagggcgctggtattttctggatatacgggaccgattacatttgagtcattctccagtagagtcgtaggacaaccattagagggaattctggcaatttggcgtaatttatgggaagatggccgcgatctagctagtcacgccttagcatatactcgtgtccagttaaaatctgctcaagaagccctaaaacaagccgagcgcagtcgcttaccgtgataa

SEQ ID NO: 70 - protein, 297 aa, Artificial Sequence
  variant 261745
MNKLGVHALVWEAGWSRDECARAIARTAETGFDFIEVPALDPASIDAEFTRRELEKHGLGVTFSLGLDAQCDISSGDPERAARGKAKLKDVLRVARDCGATHVCGPLYSAFQKYAVPTTARGVAMAADILGQVADTAAQYGITLGLEVVNRYETHVLNTASQGVELIERIGRPNVKVHLDTYHMNIEESDIMSAIRDTADRLGYFHIGDSHRGYLGSGNVDWTAVFRALVFSGYTGPITFESFSSRVVGQPLEGILAIWRNLWEDGRDLASHALAYTRVQLKSAQEALKQAERSRLP

SEQ ID NO: 71 - DNA, 897 bp, Artificial Sequence
  coding sequence for variant 261746
atgaataagttaggtgtgcacgcattagtttgggaagcgggttggagtcgtgatgagtgtgctcgtgccatcgcacgcaccgcggaaacgggatttgacttcattgaagtcccagcgttagatccggcaagcattgatgcagattttactcgcagagagttagaaaaatatgggttgggagtaaccttttcgcttggactcgatgcgcaaacagacattagttctggtgatccggaacgcgcagcgcggggtaaagctaaattaaaagatgtcttacgtgtagcccgggattgtggagcgactcatgtctgtggaattctctatagtgcatttcaaaaatatgcagttcctacgaccgcaagaggtgtcgccatggccgcggacattttaggacaggtagctgatactgcagcacaatacggtattactttggggttagaagtcgttaaccgttatgagacaaatgtattgaacaccgcgtcacagggtgttgaacttattgagcgtattggtcgtcccaacgtaaaagtgcatttagatacgtatcacatgaatattgaagagagcgatattatgagcgcgatcagagatacgggagacaggctagggtatttccatattggcgaatctcatcgtggttacctgggttccggaaacgtcgactttactgccgtatttagggcgctggtattttctggatatacgggaccgattacatttgagtcattctccagtagagtcgtaggacaaccattagagggaattctggcaatttggcgtaatttatgggaagatggccgcgatctagctagtcacgccttagcatatactcgtgtccagttaaaatctgctcaagaagccctaaaacaagccgagcgcagtcgcttaccgtgataa

SEQ ID NO: 72 - protein, 297 aa, Artificial Sequence
  variant 261746
MNKLGVHALVWEAGWSRDECARAIARTAETGFDFIEVPALDPASIDADFTRRELEKYGLGVTFSLGLDAQTDISSGDPERAARGKAKLKDVLRVARDCGGTHVCGILYSAFQKYAVPTTARGVAMAADILGQVADTAAQYGITLGLEVVNRYETNVLNTASQGVELIERIGRPNVKVHLDTYHMNIEESDIMSAIRDTGDRLGYFHLGESHRGYLGSGNVDFTAVFRALRFSGYTGPITFESFSSRVVGQPLEGILAIWRNLWEDGRDLASHALAYTRVQLKSAQEALKQAERSRLP

SEQ ID NO: 73 - DNA, 897 bp, Artificial Sequence
  coding sequence for variant 261747
atgaataagttaggtgtgcacgcattagtttgggaagcgggttggagtcgtgatgagtgtgctcgtgccatcgcacgcaccgcggaaacgggatttgacttcattgaagtcccagcgttagatccgagaagcattgatgcagagtttactcgcagagagttagaaaaacatgggttgggagtaaccttttcgcttggactcgatgcgcaaacagacattagttctggtgatccggaacgcgcagcgcggggtaaagctaaattaaaagatgtcttacgtgtagcccgggattgtggagcgactcatgtctgtggaattctctatagtgcatttcaaaaatatgcagttcctacgaccgcaagaggtgtcgccatggccgcggacattttaggacaggtagctgatactgcagcacaatacggtattactttggggttagaagtcgttaaccgttatgagacaaatgtattgaacaccgcgtcacagggtgttgaacttattgagcgtattggtcgtcccaacgtaaaagtgcatttagatacgtatcacatgaatattgaagagagcgatattatgagcgcgatcagagatacggcagacaggctagggtatttccatattggcgattctcatcgtggttacctgggttccggaaacgtcgactttactgccgtatttagggcgctggtattttctggatatacgggaccgattacatttgagtcattctccagtagagtcgtaggacaaccattagagggaattctggcaatttggcgtaatttatgggaagatggccgcgatctagctagtcacgccttagcatttactcgtgtccagttaaaatctgctcaagaagccctaaaacaagccgagcgcagtcgcttaccgtgataa

SEQ ID NO: 74 - protein, 297 aa, Artificial Sequence
  variant 261747
MNKLGVHALVWEAGWSRDECARAIARTAETGFDFIEVPALDPRSIDAEFTRRELEKHGLGVTFSLGLDAQTDISSGDPERAARGKAKLKDVLRVARDCGATHVCGILYSAFQKYAVPTTARGVAMAADILGQVADTAAQYGITLGLEVVNRYETNLLNTASQGVELIERIGRPNVKVHLDTYHANIEESDIMSAIRDTADRLGYFHIGDSHRGYLGSGNVDFTAVFRALVFSGYTGPLTFESFSSRVVGQPLEGILAIWRNLWEDGRDLASHALAFTRVQLKSAQEALKQAERSRLP

SEQ ID NO: 75 - DNA, 897 bp, Artificial Sequence
  coding sequence for variant 261748
atgaataagttaggtgtgcacgcattagtttgggaagcgggttggagtcgtgatgagtgtgctcgtgccatcgcacgcaccgcggaaacgggatttgacttcattgaagtcccagcgttagatccggcaagcattgatgcagagtttactcgcagagagttagaaaaatatgggttgggagtaaccttttcgcttggactcgatgcgcaaacagacattagttctggtgatccggaacgcgcagcgcggggtaaagctaaattaaaagatgtcttacgtgtagcccgggattgtggagcgactcatgtctgtggaattctctatagtgcatttcaaaaatatgcagttcctacgacccgtagaggtgtcgccatggccgcggacattttaggacaggtagctgatactgcagcacaatacggtattactttggggttagaagtcgttaaccgttatgagacaaatgtattgaacaccgcgtcacagggtgttgaacttattgagcgtattggtcgtcccaacgtaaaagtgcatttagatacgtatcacatgaatattgaagagagcgatattatgagcgcgatcagagatacgggagacaggctagggtatttccatattggcgaatctcatcgtggttacctgggttccggaaacgtcgactttactgccgtatttagggcgctggtattttctggatatacgggaccgattacatttgagtcattctccagtagagtcgtaggacaaccattagagggaattctggcaatttggcgtaatttatgggaagattcacgcgatctagctagtcacgccttagcatttactcgtgtccagttaaaatctgctcaagaagccctaaaacaagccgagcgcagtcgcttaccgtgataa

SEQ ID NO: 76 - protein, 297 aa, Artificial Sequence
  variant 261748
MNKLGVHALVWEAGWSRDECARAIARTAETGFDFIEVPALDPASIDAEFTRRELEKYGLGVTFSLGLDAQTDISSGDPERAARGKAKLKDVLRVARDCGATHVCGILYSAFQKYAVPTTRRGVAMAADILGQVADTAAQYGITLGLEVVNRYETYVLNTASQGVELIERIGRPNVKVHLDTYHMNIEESDIMSAIRDTGDRLGYFHIGESHRGYLGSGNLDFTAVFRALVFSGYTGPITVESFSSRVVGQPLEGILAIWRNLWEDSRDLASHALAFTRVQLKSAQEALKQAERSRLP

SEQ ID NO: 77 - DNA, 897 bp, Artificial Sequence
  coding sequence for variant 261749
atgaataagttaggtgtgcacgcattagtttgggaagcgggttggagtcgtgatgagtgtgctcgtgccatcgcacgcaccgcggaaacgggatttgacttcattgaagtcccagcgttagatccgagaagcattgatgcagagtttactcgcagagagttagaaaaacatgggttgggagtaaccttttcgcttggactcgatgcgcaaacagacattagttctggtgatccggaacgcgcagcgcggggtaaagctaaattaaaagatgtcttacgtgtagcccgggattgtggagcgactcatgtctgtggaattctctatagtgcatttcaaaaatatgcagttcctacgacccgtagaggtgtcgccatggccgcggacattttaggacaggtagctgatactgcagcacaatacggtattactttggggttagaagtcgttaaccgttatgagacaaatgtattgaacaccgcgtcacagggtgttgaacttattgagcgtattggtcgtcccaacgtaaaagtgcatttagatacgtatcacatgaatattgaagagagcgatattatgagcgcgatcagagatacggcagacaggctagggtatttccatattggcgattctcatcgtggttacctgggttccggaaacgtcgactttactgccgtatttagggcgctggtattttctggatatacgggaccgattacatttgagtcattctccagtagagtcgtaggacaaccattagagggaattctggcaatttggcgtaatttatgggaagattcacgcgatctagctagtcacgccttagcatttactcgtgtccagttaaaatctgctcaagaagccctaaaacaagccgagcgcagtcgcttaccgtgataa

SEQ ID NO: 78 - protein, 297 aa, Artificial Sequence
  variant 261749
MNKLGVHALVWEAGWSRDECARAIARTAETGFDFIEVPALDPRSIDAEFTRRELEKHGLGVTFSLGLDAQTDISSGDPERAARGKAKLKDVLRVARDCGATHVCGILYSAFQKYAVPTTRRGVAMAADILGQVADTAAQYGITLGLEVVNRYETNVLNTASQGVELIERIGRPNVKLHLDTYHMNIEESDIMSAIRDTADRLGYFHIGDSHRGYLGSGNVDFTAIFRALVFSGYTGPITLESFSSRVVGQPLEGILAIWRNLWEDSRDLASHALAFTRVQLKSAQEALKQAERSRLP

SEQ ID NO: 79 - DNA, 897 bp, Artificial Sequence
  coding sequence for variant 261750
atgaataagttaggtgtgcacgcattagtttgggaagcgggttggagtcgtgatgagtgtgctcgtgccatcgcacgcaccgcggaaacgggatttgacttcattgaagtcccagcgttagatccgagaagcattgatgcagattttactcgcagagagttagaaaaacatgggttgggagtaaccttttcgcttggactcgatgcgcaatgcgacattagttctggtgatccggaacgcgcagcgcggggtaaagctaaattaaaagatgtcttacgtgtagcccgggattgtggagcgactcatgtctgtggaattctctatagtgcatttcaaaaatatgcagttcctacgacccgtagaggtgtcgccatggccgcggacattttaggacaggtagctgatactgcagcacaatacggtattactttggggttagaagtcgttaaccgttatgagacaaatgtattgaacaccgcgtcacagggtgttgaacttattgagcgtattggtcgtcccaacgtaaaagtgcatttagatacgtatcacatgaatattgaagagagcgatattatgagcgcgatcagagatacgggagacaggctagggtatttccatattggcgaatctcatcgtggttacctgggttccggaaacgtcgactttactgccgtatttagggcgctggtattttctggatatacgggaccgattacatttgagtcattctccagtagagtcgtaggacaaccattagagggaattctggcaatttggcgtaatttatgggaagatggccgcgatctagctagtcacgccttagcatatactcgtgtccagttaaaatctgctcaagaagccctaaaacaagccgagcgcagtcgcttaccgtgataa

SEQ ID NO: 80 - protein, 297 aa, Artificial Sequence
  variant 261750
MNKLGVHALVWEAGWSRDECARAIARTAETGFDFVEVPALDPRSIDADFTRRELEKHGLGVTFSLGLDAQCDISSGDPERAARGKAKLKDVLRVARDCGATHVCGILYSAFQKYAVPTTRRGVAMAADILGQVADTAAQYGVTLGLEVVNRYETNVLNTASQGVELIERIGRPNVKVHLDTYHMNIEESDIMSAIRDTGDRLGYFHIGESHRGYLGSGNVDFTAVFRALVFSGYTGPITFESFSSRVVGQPLEGILAIWRNLWEDGRDLASHGLAYTRVQLKSAQEALKQAERSRLP

SEQ ID NO: 81 - DNA, 897 bp, Artificial Sequence
  coding sequence for variant 261751
atgaataagttaggtgtgcacgcattagtttgggaagcgggttggagtcgtgatgagtgtgctcgtgccatcgcacgcaccgcggaaacgggatttgacttcattgaagtcccagcgttagatccggcaagcattgatgcagattttactcgcagagagttagaaaaacatgggttgggagtaaccttttcgcttggactcgatgcgcaatgcgacattagttctggtgatccggaacgcgcagcgcggggtaaagctaaattaaaagatgtcttacgtgtagcccgggattgtggagcgactcatgtctgtggaattctctatagtgcatttcaaaaatatgcagttcctacgacccgtagaggtgtcgccatggccgcggacattttaggacaggtagctgatactgcagcacaatacggtattactttggggttagaagtcgttaaccgttatgagacaaatgtattgaacaccgcgtcacagggtgttgaacttattgagcgtattggtcgtcccaacgtaaaagtgcatttagatacgtatcacatgaatattgaagagagcgatattatgagcgcgatcagagatacgggagacaggctagggtatttccatattggcgaatctcatcgtggttacctgggttccggaaacgtcgactttactgccgtatttagggcgctggtattttctggatatacgggaccgattacatttgagtcattctccagtagagtcgtaggacaaccattagagggaattctggcaatttggcgtaatttatgggaagatggccgcgatctagctagtcacgccttagcatttactcgtgtccagttaaaatctgctcaagaagccctaaaacaagccgagcgcagtcgcttaccgtgataa

SEQ ID NO: 82 - protein, 297 aa, Artificial Sequence
  variant 261751
MNKLGVHALVWEAGWSRDECARAIARTAETGFDFIEVPALDPASIDADFTRRELEKHGLGVTFSLGLDAQCDISSGDPERAARGKAKLKDVLRVARDCGATHVCGILYSAFQKYAVPTTRRGVAMAADILGQVADTAAQYGITLGLEVVNRYETNVLNTASQGVELIERIGRPNVKVHLDTYHMNIEESDIMSAIRDTGDRLGYFHIGESHRGYLGTGHVDFTAVFRALVFSGYTGPLTFESFSSRVVGQPLEGILAIWRNLWEDGRDLASHALAFTRVQLKSAQEALKQAERSRLP

SEQ ID NO: 83 - DNA, 897 bp, Artificial Sequence
  coding sequence for variant 261752
atgaataagttaggtgtgcacgcattagtttgggaagcgggttggagtcgtgatgagtgtgctcgtgccatcgcacgcaccgcggaaacgggatttgacttcattgaagtcccagcgttagatccgagaagcattgatgcagattttactcgcagagagttagaaaaacatgggttgggagtaaccttttcgcttggactcgatgcgcaatgcgacattagttctggtgatccggaacgcgcagcgcggggtaaagctaaattaaaagatgtcttacgtgtagcccgggattgtggagcgactcatgtctgtggaattctctatagtgcatttcaaaaatatgcagttcctacgaccgcaagaggtgtcgccatggccgcggacattttaggacaggtagctgatactgcagcacaatacggtattactttggggttagaagtcgttaaccgttatgagacaaatgtattgaacaccgcgtcacagggtgttgaacttattgagcgtattggtcgtcccaacgtaaaagtgcatttagatacgtatcacatgaatattgaagagagcgatattatgagcgcgatcagagatacgggagacaggctagggtatttccatattggcgattctcatcgtggttacctgggttccggaaacgtcgactttactgccgtatttagggcgctggtattttctggatatacgggaccgattacatttgagtcattctccagtagagtcgtaggacaaccattagagggaattctggcaatttggcgtaatttatgggaagatggccgcgatctagctagtcacgccttagcatatactcgtgtccagttaaaatctgctcaagaagccctaaaacaagccgagcgcagtcgcttaccgtgataa

SEQ ID NO: 84 - protein, 297 aa, Artificial Sequence
  variant 261752
MNKLGVHALVWEAGWSRDECARAIARTAETGFDFIEVPALDPRSIDADFTRRELEKHGLGVTFSLGLDAQCDISSGDPERAARGKAKLKDVLRVARDCGATHVCGILYSAFQKYAVPTTARGVAMAADILGQVADTAAQYGITLGLEVVNRFETNVLNTASQGVELIERIGRPNVKVHLDTYHMNIEESDIMSAIRDTGDRLGYFHIGDSHRGYLGSGNLDFTAVFRALVFSGYTGPITFESFSSRVVGQPLEGILAIWRNLWEDGRDLASHALAYLRVQLKSAQEALKQAERSRLP

SEQ ID NO: 85 - DNA, 897 bp, Artificial Sequence
  coding sequence for variant 261753
atgaataagttaggtgtgcacgcattagtttgggaagcgggttggagtcgtgatgagtgtgctcgtgccatcgcacgcaccgcggaaacgggatttgacttcattgaagtcccagcgttagatccggcaagcattgatgcagagtttactcgcagagagttagaaaaatatgggttgggagtaaccttttcgcttggactcgatgcgcaatgcgacattagttctggtgatccggaacgcgcagcgcggggtaaagctaaattaaaagatgtcttacgtgtagcccgggattgtggagcgactcatgtctgtggaattctctatagtgcatttcaaaaatatgcagttcctacgacccgtagaggtgtcgccatggccgcggacattttaggacaggtagctgatactgcagcacaatacggtattactttggggttagaagtcgttaaccgttatgagacaaatgtattgaacaccgcgtcacagggtgttgaacttattgagcgtattggtcgtcccaacgtaaaagtgcatttagatacgtatcacatgaatattgaagagagcgatattatgagcgcgatcagagatacggcagacaggctagggtatttccatattggcgattctcatcgtggttacctgggttccggaaacgtcgactttactgccgtatttagggcgctggtattttctggatatacgggaccgattacatttgagtcattctccagtagagtcgtaggacaaccattagagggaattctggcaatttggcgtaatttatgggaagattcacgcgatctagctagtcacgccttagcatatactcgtgtccagttaaaatctgctcaagaagccctaaaacaagccgagcgcagtcgcttaccgtgataa

SEQ ID NO: 86 - protein, 297 aa, Artificial Sequence
  variant 261753
MNKLGVHALVWEAGWSRDECARAIARTAETGFDFIELPALDPASIDAEFTRRELEKYGLGVTFSLGLDAQCDISSGDPERAARGKAKLKDVLRVARDCGATHVCGILYSAFQKYAVPTTRRGVAMAADILGQVADTAAQYGVTLGLEVVNRYETNLLNTASQGVELIERIGRPNVKVHLDTYHMNIEESDIMSAIRDTADRLGYFHIGDSHRGYLGSGNVDFTAVFRALVFSGYTGPITFESFSSRVVGQPLEGILAIWRNLWEDSRDLASHALAYTRVQLKSAQEALKQAERSRLP

SEQ ID NO: 87 - DNA, 897 bp, Artificial Sequence
  coding sequence for variant 261754
atgaataagttaggtgtgcacgcattagtttgggaagcgggttggagtcgtgatgagtgtgctcgtgccatcgcacgcaccgcggaaacgggatttgacttcattgaagtcccagcgttagatccggcaagcattgatgcagagtttactcgcagagagttagaaaaatatgggttgggagtaaccttttcgcttggactcgatgcgcaaacagacattagttctggtgatccggaacgcgcagcgcggggtaaagctaaattaaaagatgtcttacgtgtagcccgggattgtggagcgactcatgtctgtggaattctctatagtgcatttcaaaaatatgcagttcctacgaccgcaagaggtgtcgccatggccgcggacattttaggacaggtagctgatactgcagcacaatacggtattactttggggttagaagtcgttaaccgttatgagacaaatgtattgaacaccgcgtcacagggtgttgaacttattgagcgtattggtcgtcccaacgtaaaagtgcatttagatacgtatcacatgaatattgaagagagcgatattatgagcgcgatcagagatacggcagacaggctagggtatttccatattggcgattctcatcgtggttacctgggttccggaaacgtcgactttactgccgtatttagggcgctggtattttctggatatacgggaccgattacatttgagtcattctccagtagagtcgtaggacaaccattagagggaattctggcaatttggcgtaatttatgggaagattcacgcgatctagctagtcacgccttagcatatactcgtgtccagttaaaatctgctcaagaagccctaaaacaagccgagcgcagtcgcttaccgtgataa

SEQ ID NO: 88 - protein, 297 aa, Artificial Sequence
  variant 261754
MNKLGVHALVWEAGWSRDECARAIARTAETGFDFIEVPALDPASIDAEFTRRELEKYGLGVTFSLGLDAQTDISSGDPERAARGKAKLKDVLRVARDCGATHVCGILYSAFQKYAVPTTARGVAMAADILGQVADTAAQYGITLGLEVVNRYETNVLNTASQGVELIERIGRPNVKVHLDTYHMNIEESDIMSAIRDTADRLGYFHIGDSHRGYLGSGNVDFTAVFRALVFSGYTGPITMECFSSRVVGQPLEGILAIWRNLWEDSRDVASHALAYTRVQLKSAQEALKQAERSRLP

SEQ ID NO: 89 - DNA, 897 bp, Artificial Sequence
  coding sequence for variant 277285
atgaataagttaggtgtgcacgcattagtttgggaagcgggttggagtcgtgatgagtgtgctcgtgccatcgcacgcaccgcggaaacgggatttgacttcattgaagtcccagcgttagatccggcaagcattgatgcagagtttactcgcagagagttagaacgccatgggttgggagtaaccttttcgcttggactcgatgcgcaaacagacattagttctggtgatccggaacgcgcagcgcggggtaaagctaaattaaaagatgtcttacgtgtagcccgggattgtggagcgactcatgtctgtggaattctctatagtgcatttcaaaaaaatgcagttcctacgacccgtgcgggtgtcgccatggccgcggacattttaggacaggtagctgatactgcagcacaatacggtattactttggggttagaagtcgttaaccgttatgagtcaaatgtattgaacaccgcgtcacagggtgttgaactttgcgagcgtattggtcgtcccaacgtaaaagtgcatttagatacgtatcacatgaatattgaagagagcgatattatgagcgcgatcagagatacgggagacaggctagggtatttccatattggcgattctcatcgtggttacctgggttccggaaacgtcgactttactgccgtatttagggcgctggtattttctggatatacgggaccgattacatttgagtcattctccagtagagtcgtaggacaaccattagagggaattctggcaatttggcgtaatttatgggaagattcccgcgatctagctagtcacgccttagcatatactcgtgtccagttaaaatctgctcaagaagccctaaaacaagccgagcgcagtcgcttaccgtgataa

SEQ ID NO: 90 - protein, 297 aa, Artificial Sequence
  variant 277285
MNKLGVHALVWEAGWSRDECARAIARTAETGFDFIEVPALDPASIDAEFTRRELERHGLGVTFSLGLDAQTDISSGDPERAARGKAKLKDVLRVARDCGATHVCGILYSAFQKNAVPTTRAGVAMAADILGQVADTAAQYGITLGLEVVNRYESNVLNTASQGVELCERIGRPNVKVHLDTYHMNIEESDIMSAIRDTGDRLGYFHIGDSHRGYLGSGNVDFTAVFRALVFSGYTGPITFESFSSRVVGQPLEGILAIWRNLWEDSRDLASHALAYTRVQLKSAQEALKQAERSRLP

SEQ ID NO: 91 - DNA, 897 bp, Artificial Sequence
  coding sequence for variant 277286
atgaataagttaggtgtgcacgcattagtttgggaagcgggttggagtcgtgatgagtgtgctcgtgccatcgcacgcaccgcggaaacgggatttgacttcattgaagtcccagcgttagatccggcaagcattgatgcagagtttactcgcagagagttagaacgccatgggttgggagtaaccttttcgcttggactcgatgcgcaaacagacattagttctggtgatccggaacgcgcagcgcggggtaaagctaaattagacgatgtcttacgtgtagcccgggattgtggagcgactcatgtctgtggaattctctatagtgcatttcaaaaaaatgcagttcctacgacccgtgcgggtgtcgccatggccgcggacattttaggacaggtagctgatactgcagcacaatacggtattactttggggttagaagtcgttaaccgttatgagacaaatgtattgaacaccgcgtcacagggtgttgaactttgcgagcgtattggtcgtcccaacgtaaaagtgcatttagatacgtatcacatgaatattgaagagagcgatattatgagcgcgatcagagatacgggagacaggctagggtatttccatattggcgattctcatcgtggttacctgggttccggaaacgtcgactttactgccgtatttagggcgctggtattttctggatatacgggaccgattacatttgagtcattctccagtagagtcgtaggacaaccattagagggaattctggcaatttggcgtaatttatgggaagattcccgcgatctagctagtcacgccttagcatatactcgtgtccagttaaaatctgctcaagaagccctaaaacaagccgagcgcagtcgcttaccgtgataa

SEQ ID NO: 92 - protein, 297 aa, Artificial Sequence
  variant 277286
MNKLGVHALVWEAGWSRDECARAIARTAETGFDFIEVPALDPASIDAEFTRRELERHGLGVTFSLGLDAQTDISSGDPERAARGKAKLDDVLRVARDCGATHVCGILYSAFQKNAVPTTRAGVAMAADILGQVADTAAQYGITLGLEVVNRYETNVLNTASQGVELCERIGRPNVKVHLDTYHMNIEESDIMSAIRDTGDRLGYFHIGDSHRGYLGSGNVDFTAVFRALVFSGYTGPITFESFSSRVVGQPLEGILAIWRNLWEDSRDLASHALAYTRVQLKSAQEALKQAERSRLP

SEQ ID NO: 93 - DNA, 897 bp, Artificial Sequence
  coding sequence for variant 277287
atgaataagttaggtgtgcacgcattagtttgggaagcgggttggagtcgtgatgagtgtgctcgtgccatcgcacgcaccgcggaaacgggatttgacttcattgaagtcccagcgttagatccggcaagcattgatgcagagtttactcgcagagagttagaacgccatgggttgggagtaaccttttcgcttggactcgatgcgcaaacagacattagttctggtgatccggaacgcgcagcgcggggtaaagctaaattagacgatgtcttacgtgtagcccgggattgtggagcgactcatgtctgtggaattctctatagtgcatttcaaaaaaatgcagttcctacgacccgtgcgggtgtcgccatggccgcggacattttaggacaggtagctgatactgcagcacaatacggtattactttggggttagaagtcgttaaccgttatgagtcaaatgtattgaacaccgcgtcacagggtgttgaacttattgagcgtattggtcgtcccaacgtaaaagtgcatttagatacgtatcacatgaatattgaagagagcgatattatgagcgcgatcagagatacgggagacaggctagggtatttccatattggcgattctcatcgtggttacctgggttccggaaacgtcgactttactgccgtatttagggcgctggtattttctggatatacgggaccgattacatttgagtcattctccagtagagtcgtaggacaaccattagagggaattctggcaatttggcgtaatttatgggaagattcccgcgatctagctagtcacgccttagcatatactcgtgtccagttaaaatctgctcaagaagccctaaaacaagccgagcgcagtcgcttaccgtgataa

SEQ ID NO: 94 - protein, 297 aa, Artificial Sequence
  variant 277287
MNKLGVHALVWEAGWSRDECARAIARTAETGFDFIEVPALDPASIDAEFTRRELERHGLGVTFSLGLDAQTDISSGDPERAARGKAKLDDVLRVARDCGATHVCGILYSAFQKNAVPTTRAGVAMAADILGQVADTAAQYGITLGLEVVNRYESNVLNTASQGVELIERIGRPNVKVHLDTYHMNIEESDIMSAIRDTGDRLGYFHIGDSHRGYLGSGNVDFTAVFRALVFSGYTGPITFESFSSRVVGQPLEGILAIWRNLWEDSRDLASHALAYTRVQLKSAQEALKQAERSRLP

SEQ ID NO: 95 - DNA, 897 bp, Artificial Sequence
  coding sequence for variant 277288
atgaataagttaggtgtgcacgcattagtttgggaagcgggttggagtcgtgatgagtgtgctcgtgccatcgcacgcaccgcggaaacgggatttgacttcattgaagtcccagcgttagatccggcaagcattgatgcagagtttactcgcagagagttagaacgccatgggttgggagtaaccttttcgcttggactcgatgcgcaaacagacattagttctggtgatccggaacgcgcagcgcggggtaaagctaaattaaaagatgtcttacgtgtagcccgggattgtggagcgactcatgtctgtggaattctctatagtgcatttcaaaaaaatgcagttcctacgacccgtgcgggtgtcgccatggccgcggacattttaggacaggtagctgatactgcagcacaatacggtattactttggggttagaagtcgttaaccgttatgagacaaatgtattgaacaccgcgtcacagggtgttgaactttgcgagcgtattggtcgtcccaacgtaaaagtgcatttagatacgtatcacatgaatattgaagagagcgatattatgagcgcgatcagagatacgggagacaggctagggtatttccatattggcgattctcatcgtggttacctgggttccggaaacgtcgactttactgccgtatttagggcgctggtattttctggatatacgggaccgattacatttgagtcattctccagtagagtcgtaggacaaccattagagggaattctggcaatttggcgtaatttatgggaagattcccgcgatctagctagtcacgccttagcatatactcgtgtccagttaaaatctgctcaagaagccctaaaacaagccgagcgcagtcgcttaccgtgataa

SEQ ID NO: 96 - protein, 297 aa, Artificial Sequence
  variant 277288
MNKLGVHALVWEAGWSRDECARAIARTAETGFDFIEVPALDPASIDAEFTRRELERHGLGVTFSLGLDAQTDISSGDPERAARGKAKLKDVLRVARDCGATHVCGILYSAFQKNAVPTTRAGVAMAADILGQVADTAAQYGITLGLEVVNRYETNVLNTASQGVELCERIGRPNVKVHLDTYHMNIEESDIMSAIRDTGDRLGYFHIGDSHRGYLGSGNVDFTAVFRALVFSGYTGPITFESFSSRVVGQPLEGILAIWRNLWEDSRDLASHALAYTRVQLKSAQEALKQAERSRLP

SEQ ID NO: 97 - DNA, 897 bp, Artificial Sequence
  coding sequence for variant 277289
atgaataagttaggtgtgcacgcattagtttgggaagcgggttggagtcgtgatgagtgtgctcgtgccatcgcacgcaccgcggaaacgggatttgacttcattgaagtcccagcgttagatccggcaagcattgatgcagagtttactcgcagagagttagaacgccatgggttgggagtaaccttttcgcttggactcgatgcgcaaacagacattagttctggtgatccggaacgcgcagcgcggggtaaagctaaattagacgatgtcttacgtgtagcccgggattgtggagcgactcatgtctgtggaattctctatagtgcatttcaaaaaaatgcagttcctacgacccgtgcgggtgtcgccatggccgcggacattttaggacaggtagctgatactgcagcacaatacggtattactttggggttagaagtcgttaaccgttatgagacaaatgtattgaacaccgcgtcacagggtgttgaacttattgagcgtattggtcgtcccaacgtaaaagtgcatttagatacgtatcacatgaatattgaagagagcgatattatgagcgcgatcagagatacgggagacaggctagggtatttccatattggcgattctcatcgtggttacctgggttccggaaacgtcgactttactgccgtatttagggcgctggtattttctggatatacgggaccgattacatttgagtcattctccagtagagtcgtaggacaaccattagagggaattctggcaatttggcgtaatttatgggaagattcccgcgatctagctagtcacgccttagcatatactcgtgtccagttaaaatctgctcaagaagccctaaaacaagccgagcgcagtcgcttaccgtgataa

SEQ ID NO: 98 - protein, 297 aa, Artificial Sequence
  variant 277289
MNKLGVHALVWEAGWSRDECARAIARTAETGFDFIEVPALDPASIDAEFTRRELERHGLGVTFSLGLDAQTDISSGDPERAARGKAKLDDVLRVARDCGATHVCGILYSAFQKNAVPTTRAGVAMAADILGQVADTAAQYGITLGLEVVNRYETNVLNTASQGVELIERIGRPNVKVHLDTYHMNIEESDIMSAIRDTGDRLGYFHIGDSHRGYLGSGNVDFTAVFRALVFSGYTGPITFESFSSRVVGQPLEGILAIWRNLWEDSRDLASHALAYTRVQLKSAQEALKQAERSRLP

SEQ ID NO: 99 - DNA, 897 bp, Artificial Sequence
  coding sequence for variant 277290
atgaataagttaggtgtgcacgcattagtttgggaagcgggttggagtcgtgatgagtgtgctcgtgccatcgcacgcaccgcggaaacgggatttgacttcattgaagtcccagcgttagatccggcaagcattgatgcagagtttactcgcagagagttagaacgccatgggttgggagtaaccttttcgcttggactcgatgcgcaaacagacattagttctggtgatccggaacgcgcagcgcggggtaaagctaaattaaaagatgtcttacgtgtagcccgggattgtggagcgactcatgtctgtggaattctctatagtgcatttcaaaaaaatgcagttcctacgacccgtgcgggtgtcgccatggccgcggacattttaggacaggtagctgatactgcagcacaatacggtattactttggggttagaagtcgttaaccgttatgagtcaaatgtattgaacaccgcgtcacagggtgttgaacttattgagcgtattggtcgtcccaacgtaaaagtgcatttagatacgtatcacatgaatattgaagagagcgatattatgagcgcgatcagagatacgggagacaggctagggtatttccatattggcgattctcatcgtggttacctgggttccggaaacgtcgactttactgccgtatttagggcgctggtattttctggatatacgggaccgattacatttgagtcattctccagtagagtcgtaggacaaccattagagggaattctggcaatttggcgtaatttatgggaagattcccgcgatctagctagtcacgccttagcatatactcgtgtccagttaaaatctgctcaagaagccctaaaacaagccgagcgcagtcgcttaccgtgataa

SEQ ID NO: 100 - protein, 297 aa, Artificial Sequence
  variant 277290
MNKLGVHALVWEAGWSRDECARAIARTAETGFDFIEVPALDPASIDAEFTRRELERHGLGVTFSLGLDAQTDISSGDPERAARGKAKLKDVLRVARDCGATHVCGILYSAFQKNAVPTTRAGVAMAADILGQVADTAAQYGITLGLEVVNRYESNVLNTASQGVELIERIGRPNVKVHLDTYHMNIEESDIMSAIRDTGDRLGYFHIGDSHRGYLGSGNVDFTAVFRALVFSGYTGPITFESFSSRVVGQPLEGILAIWRNLWEDSRDLASHALAYTRVQLKSAQEALKQAERSRLP